European Patent Application EP 4 299 732 A2, published January 3, 2024. Title: RATS COMPRISING A HUMANIZED TRKB LOCUS. Applicant: Regeneron Pharmaceuticals, Inc. Application EP, filed November 30, 2018. The sequence listing filed with the application follows.

SEQUENCE LISTING (125 sequences)

SEQ ID NO: 1 - protein, 821 aa, Mus musculus
  REGION 1..31: note = MISC_FEATURE - Signal Peptide
  REGION 32..429: note = MISC_FEATURE - Extracellular Domain
  REGION 430..453: note = MISC_FEATURE - Transmembrane Domain
  REGION 454..821: note = MISC_FEATURE - Cytoplasmic Domain
MSPWLKWHGPAMARLWGLCLLVLGFWRASLACPTSCKCSSARIWCTEPSPGIVAFPRLEPNSVDPENITEILIANQKRLEIINEDDVEAYVGLRNLTIVDSGLKFVAYKAFLKNSNLRHINFTRNKLTSLSRRHFRHLDLSDLILTGNPFTCSCDIMWLKTLQETKSSPDTQDLYCLNESSKNMPLANLQIPNCGLPSARLAAPNLTVEEGKSVTLSCSVGGDPLPTLYWDVGNLVSKHMNETSHTQGSLRITNISSDDSGKQISCVAENLVGEDQDSVNLTVHFAPTITFLESPTSDHHWCIPFTVRGNPKPALQWFYNGAILNESKYICTKIHVTNHTEYHGCLQLDNPTHMNNGDYTLMAKNEYGKDERQISAHFMGRPGVDYETNPNYPEVLYEDWTTPTDIGDTTNKSNEIPSTDVADQSNREHLSVYAVVVIASVVGFCLLVMLLLLKLARHSKFGMKGPASVISNDDDSASPLHHISNGSNTPSSSEGGPDAVIIGMTKIPVIENPQYFGITNSQLKPDTFVQHIKRHNIVLKRELGEGAFGKVFLAECYNLCPEQDKILVAVKTLKDASDNARKDFHREAELLTNLQHEHIVKFYGVCVEGDPLIMVFEYMKHGDLNKFLRAHGPDAVLMAEGNPPTELTQSQMLHIAQQIAAGMVYLASQHFVHRDLATRNCLVGENLLVKIGDFGMSRDVYSTDYYRVGGHTMLPIRWMPPESIMYRKFTTESDVWSLGVVLWEIFTYGKQPWYQLSNNEVIECITQGRVLQRPRTCPQEVYELMLGCWQREPHTRKNIKSIHTLLQNLAKASPVYLDILG

SEQ ID NO: 2 - protein, 821 aa, Rattus norvegicus
  REGION 1..31: note = MISC_FEATURE - Signal Peptide
  REGION 32..429: note = MISC_FEATURE - Extracellular Domain
  REGION 430..453: note = MISC_FEATURE - Transmembrane Domain
  REGION 454..821: note = MISC_FEATURE - Cytoplasmic Domain
MSPWPRWHGPAMARLWGLCLLVLGFWRASLACPMSCKCSTTRIWCTEPSPGIVAFPRLEPNSIDPENITEILIANQKRLEIINEDDVEAYVGLKNLTIVDSGLKFVAYKAFLKNGNLRHINFTRNKLTSLSRRHFRHLDLSDLILTGNPFTCSCDIMWLKTLQETKSSPDTQDLYCLNESSKNTPLANLQIPNCGLPSARLAAPNLTVEEGKSVTISCSVGGDPLPTLYWDVGNLVSKHMNETSHTQGSLRITNISSDDSGKQISCVAENLVGEDQDSVNLTVHFAPTITFLESPTSDHHWCIPFTVRGNPKPALQWFYNGAILNESKYICTKIHVTNHTEYHGCLQLDNPTHMNNGDYTLMAKNEYGKDERQISAHFMGRPGVDYETNPNYPEVLYEDWTTPTDIGDTTNKSNEIPSTDVADQTNREHLSVYAVVVIASVVGFCLLVMLLLLKLARHSKFGMKGPASVISNDDDSASPLHHISNGSNTPSSSEGGPDAVIIGMTKIPVIENPQYFGITNSQLKPDTFVQHIKRHNIVLKRELGEGAFGKVFLAECYNLCPEQDKILVAVKTLKDASDNARKDFHREAELLTNLQHEHIVKFYGVCVEGDPLIMVFEYMKHGDLNKFLRAHGPDAVLMAEGNPPTELTQSQMLHIAQQIAAGMVYLASQHFVHRDLATRNCLVGENLLVKIGDFGMSRDVYSTDYYRVGGHTMLPIRWMPPESIMYRKFTTESDVWSLGVVLWEIFTYGKQPWYQLSNNEVIECITQGRVLQRPRTCPQEVYELMLGCWQREPHTRKNIKNIHTLLQNLAKASPVYLDILG

SEQ ID NO: 3 - protein, 838 aa, Homo sapiens
  REGION 1..31: note = MISC_FEATURE - Signal Peptide
  REGION 32..430: note = MISC_FEATURE - Extracellular Domain
  REGION 431..454: note = MISC_FEATURE - Transmembrane Domain
  REGION 455..838: note = MISC_FEATURE - Cytoplasmic Domain
MSSWIRWHGPAMARLWGFCWLVVGFWRAAFACPTSCKCSASRIWCSDPSPGIVAFPRLEPNSVDPENITEIFIANQKRLEIINEDDVEAYVGLRNLTIVDSGLKFVAHKAFLKNSNLQHINFTRNKLTSLSRKHFRHLDLSELILVGNPFTCSCDIMWIKTLQEAKSSPDTQDLYCLNESSKNIPLANLQIPNCGLPSANLAAPNLTVEEGKSITLSCSVAGDPVPNMYWDVGNLVSKHMNETSHTQGSLRITNISSDDSGKQISCVAENLVGEDQDSVNLTVHFAPTITFLESPTSDHHWCIPFTVKGNPKPALQWFYNGAILNESKYICTKIHVTNHTEYHGCLQLDNPTHMNNGDYTLIAKNEYGKDEKQISAHFMGWPGIDDGANPNYPDVIYEDYGTAANDIGDTTNRSNEIPSTDVTDKTGREHLSVYAVVVIASVVGFCLLVMLFLLKLARHSKFGMKDFSWFGFGKVKSRQGVGPASVISNDDDSASPLHHISNGSNTPSSSEGGPDAVIIGMTKIPVIENPQYFGITNSQLKPDTFVQHIKRHNIVLKRELGEGAFGKVFLAECYNLCPEQDKILVAVKTLKDASDNARKDFHREAELLTNLQHEHIVKFYGVCVEGDPLIMVFEYMKHGDLNKFLRAHGPDAVLMAEGNPPTELTQSQMLHIAQQIAAGMVYLASQHFVHRDLATRNCLVGENLLVKIGDFGMSRDVYSTDYYRVGGHTMLPIRWMPPESIMYRKFTTESDVWSLGVVLWEIFTYGKQPWYQLSNNEVIECITQGRVLQRPRTCPQEVYELMLGCWQREPHMRKNIKGIHTLLQNLAKASPVYLDILG

SEQ ID NO: 4 - protein, 822 aa, synthetic construct
  REGION 1..822: note = Synthetic
  REGION 1..31: note = MISC_FEATURE - Signal Peptide
  REGION 1..31: note = MISC_FEATURE - Mouse Sequence
  REGION 32..430: note = MISC_FEATURE - Extracellular Domain
  REGION 32..432: note = MISC_FEATURE - Human Sequence
  REGION 431..454: note = MISC_FEATURE - Transmembrane Domain
  REGION 433..822: note = MISC_FEATURE - Mouse Sequence
  REGION 455..822: note = MISC_FEATURE - Cytoplasmic Domain
MSPWLKWHGPAMARLWGLCLLVLGFWRASLACPTSCKCSASRIWCSDPSPGIVAFPRLEPNSVDPENITEIFIANQKRLEIINEDDVEAYVGLRNLTIVDSGLKFVAHKAFLKNSNLQHINFTRNKLTSLSRKHFRHLDLSELILVGNPFTCSCDIMWIKTLQEAKSSPDTQDLYCLNESSKNIPLANLQIPNCGLPSANLAAPNLTVEEGKSITLSCSVAGDPVPNMYWDVGNLVSKHMNETSHTQGSLRITNISSDDSGKQISCVAENLVGEDQDSVNLTVHFAPTITFLESPTSDHHWCIPFTVKGNPKPALQWFYNGAILNESKYICTKIHVTNHTEYHGCLQLDNPTHMNNGDYTLIAKNEYGKDEKQISAHFMGWPGIDDGANPNYPDVIYEDYGTAANDIGDTTNRSNEIPSTDVTDKTGREHLSVYAVVVIASVVGFCLLVMLLLLKLARHSKFGMKGPASVISNDDDSASPLHHISNGSNTPSSSEGGPDAVIIGMTKIPVIENPQYFGITNSQLKPDTFVQHIKRHNIVLKRELGEGAFGKVFLAECYNLCPEQDKILVAVKTLKDASDNARKDFHREAELLTNLQHEHIVKFYGVCVEGDPLIMVFEYMKHGDLNKFLRAHGPDAVLMAEGNPPTELTQSQMLHIAQQIAAGMVYLASQHFVHRDLATRNCLVGENLLVKIGDFGMSRDVYSTDYYRVGGHTMLPIRWMPPESIMYRKFTTESDVWSLGVVLWEIFTYGKQPWYQLSNNEVIECITQGRVLQRPRTCPQEVYELMLGCWQREPHTRKNIKSIHTLLQNLAKASPVYLDILG

SEQ ID NO: 5 - protein, 822 aa, synthetic construct
  REGION 1..822: note = Synthetic
  REGION 1..31: note = MISC_FEATURE - Signal Peptide
  REGION 1..31: note = MISC_FEATURE - Rat Sequence
  REGION 32..430: note = MISC_FEATURE - Extracellular Domain
  REGION 32..432: note = MISC_FEATURE - Human Sequence
  REGION 431..454: note = MISC_FEATURE - Transmembrane Domain
  REGION 433..822: note = MISC_FEATURE - Rat Sequence
  REGION 455..822: note = MISC_FEATURE - Cytoplasmic Domain
MSPWPRWHGPAMARLWGLCLLVLGFWRASLACPTSCKCSASRIWCSDPSPGIVAFPRLEPNSVDPENITEIFIANQKRLEIINEDDVEAYVGLRNLTIVDSGLKFVAHKAFLKNSNLQHINFTRNKLTSLSRKHFRHLDLSELILVGNPFTCSCDIMWIKTLQEAKSSPDTQDLYCLNESSKNIPLANLQIPNCGLPSANLAAPNLTVEEGKSITLSCSVAGDPVPNMYWDVGNLVSKHMNETSHTQGSLRITNISSDDSGKQISCVAENLVGEDQDSVNLTVHFAPTITFLESPTSDHHWCIPFTVKGNPKPALQWFYNGAILNESKYICTKIHVTNHTEYHGCLQLDNPTHMNNGDYTLIAKNEYGKDEKQISAHFMGWPGIDDGANPNYPDVIYEDYGTAANDIGDTTNRSNEIPSTDVTDKTGREHLSVYAVVVIASVVGFCLLVMLLLLKLARHSKFGMKGPASVISNDDDSASPLHHISNGSNTPSSSEGGPDAVIIGMTKIPVIENPQYFGITNSQLKPDTFVQHIKRHNIVLKRELGEGAFGKVFLAECYNLCPEQDKILVAVKTLKDASDNARKDFHREAELLTNLQHEHIVKFYGVCVEGDPLIMVFEYMKHGDLNKFLRAHGPDAVLMAEGNPPTELTQSQMLHIAQQIAAGMVYLASQHFVHRDLATRNCLVGENLLVKIGDFGMSRDVYSTDYYRVGGHTMLPIRWMPPESIMYRKFTTESDVWSLGVVLWEIFTYGKQPWYQLSNNEVIECITQGRVLQRPRTCPQEVYELMLGCWQREPHTRKNIKNIHTLLQNLAKASPVYLDILG

SEQ ID NO: 6 - DNA, 8744 bp, Mus musculus
  source 1..8744: mol_type = other DNA
gtctggagggtgctatgctatgcgtgtgtgcgtgtgtgtgcgcgcgcgcgtgtgtgagcgtgtgtgtttttggatttcatactaattttctggagtttctgcccctgctctgcgtcagccctcacgtcacttcgccagcagtagcagaggcggcggcggcggcggccgccggttagagcccagtcgctgcttcagctgctgttgctgcttctgcagcgctctgctccctgcgcttgctacgggaggccggggaagccgcgcggacagtcctcggtggcctgggccggcactgtcctgctaccgcagttgctccccagccctgaggtgcgcaccgatatcgatattcgtgccggtttagcggttctgcgacccaaagagtccagggagatccaccgagtggtgcctggcgtataggactatgcagccgccttgtggctcggagcagcggcccgcgatgtcccagccactgtgaaccatttggtcagcgccaacctgctcagccccagcaccgacaggctcagcctctggtacgctccactccgcgggaggccaccagcaccaagcagcaagagggcgcagggaaggcctcccccctccggcgggggacgcctggctcagcgtagggacacgcactccgactgactggcactggcagctcgggatgtcgccctggctgaagtggcatggacccgccatggcgcggctctggggcttatgcctgctggtcttgggcttctggagggcctctctcgcctgcccgacgtcctgcaaatgcagttccgctaggatttggtgtactgagccttctccaggcatcgtggcattcccgaggttggaacctaacagcgttgacccggagaacatcacggaaattctcattgcaaaccagaaaaggctagaaatcatcaatgaagatgacgttgaagcttacgtggggctgagaaaccttacaattgtggattccggcttaaagtttgtggcttacaaagcgtttctgaaaaacagcaacctgcggcacataaatttcacacgaaacaagctgacgagtttgtccaggagacatttccgccaccttgacttgtctgacctgatcctgacgggtaatccgttcacgtgctcctgcgacatcatgtggctcaagactctccaggagactaaatccagccccgacactcaggatttgtactgcctcaatgagagcagcaagaacatgcccctggcgaacctgcagatacccaattgtggtctgccatctgcacgtctggctgctcctaacctcaccgtggaggaaggaaagtctgtgaccctttcctgcagtgtggggggtgacccactccccaccttgtactgggacgttgggaatttggtttccaagcacatgaatgaaacaagccacacacagggctccttaaggataacgaacatttcatctgatgacagtggaaagcaaatctcttgtgtggcagaaaaccttgtaggagaagatcaagattctgtgaacctcactgtgcattttgcgccaactatcacgtttctcgagtctccaacctcagatcaccactggtgcattccattcactgtgagaggcaaccccaagcctgcgcttcagtggttctacaatggggccatactgaatgagtccaagtacatctgtactaagatccacgtcaccaatcacacggagtaccatggctgcctccagctggataaccccactcatatgaataacggagactacaccctgatggccaagaacgagtatgggaaggatgagagacagatctccgctcacttcatgggccggcctggagtcgactacgagacaaacccaaattaccctgaagtcctctatgaagactggaccacgccaactgacattggggatactacgaacaaaagtaatgaaatcccctccacggatgttgctgaccaaagcaatcgggagcatctctcggtctatgccgtggtggtgattgcatctgtggtgggattctgcctgctggtgatgttgctcctgctcaagttggcgagacattccaagtttggcatgaaaggcccagcttcggtcatcagcaacgacgatgactctgccagccccctccaccacatctccaatgggagtaacactccatcttcttcggagggcggtcccgacgctgtcattattggaatgaccaagattcctgttattgaaaacccccagtactttggcatcaccaacagtcagctcaagccagacacatttgttcagcatatcaagagacacaacatcgttctgaagagggaacttggggaaggagccttcgggaaagttttccttgccgagtgctacaacctctgcccagagcaggataagatcctggtggctgtgaagacgctgaaggacgccagcgacaatgcacgcaaggactttcatcgggaagctgagctgctgaccaacctccagcacgagcacattgtcaagttctacggtgtctgtgtggagggcgacccactcatcatggtctttgagtacatgaagcacggggacctcaacaagttccttagggcacacgggcccgacgcagtgctgatggcagagggtaacccgcccacagagctgacgcagtcgcagatgctgcacatcgctcagcaaatcgcagcaggtatggtctacctggcgtcccaacactttgtgcaccgtgacctggccacccggaactgcctggtgggagagaacctgctggtgaaaattggggactttgggatgtcccgagatgtgtacagcaccgactactatcgggtcggtggccacacaatgttgcccatccgatggatgcctccagagagcatcatgtacaggaaattcaccaccgagagcgacgtctggagcctgggcgttgtgttgtgggagatcttcacctacggcaagcagccctggtatcagctatcgaacaatgaggtgatagagtgcatcacccagggaagagtccttcagcggcctcgaacgtgtccccaggaggtgtatgagctcatgcttggatgctggcagcgggaaccacacacccggaagaacatcaagagcatccacaccctccttcagaacttggccaaggcatctcccgtctacctggatatcctaggctagggtcctccttctgcccagaccgtccttcccaaggccctcctcagactggcctacacgacgaacctcttgactgccgctgacgtcatgaccttgctgtccttcgctctgacagtgttgacaggaccaggagcggctctttgggggaggcagtgtgtgcttctccatccacagacagtattaactcgcttctggcattgtctctttctctcccttgggtttgtttctttcttttgccccttccccttttatcattatttattcatttatttattttctggtcttcaccgcttcacggccctcagtctctccttgaccaatctggcttctgcattcctattaactgtacatagacaaaggccttaacaaacctaatttgttatatcagcagacactccagtttgcccaccacaactaacaatgccttgttgtattcctgcctttgacgtggatgaaaaaaagggaaaaaaaaatcaaacatctgacttaagctgtcacttccgatgtacagacgtggggcgtttctatggattcacttctatttattatttattaatttatttatttatcactcttcttattgttttctggtggttttaacctatgtgtgagaaggaaaagttgtgtacaatctgggaaaactttatcagtgggaaatgaaaacgagagcgagcaagcgagcaagagagggagagagagagagaagcgttaccataaaccacggcatgagcgagacagagacaagccatgggatcagtcgggagtccgttgtgcttaggaaaacccagcagccattagctgggggagcatgttcggctctgtcccccaagcacctttctgaggaggacacaggatgttgaactctgcttcacgggcagagcttctaatgacagatactggcttgcactggaaagacagttcccacgggacctggacggacaacacatcctacattcagacattgtggtcgggcacggtgacagagttgatccgtttctcaagtgttatctaccaagcttttgtgaagttccatcgaaggaggtagattcttgctcagatataatttcaggaaaacccgagtccttgacaaagacaggagacgctctcaatttggaggcaagtttctcttaccttgaactttttcagacagcaactccgcccagcccccatcttccactctcacctgtcttgtaactgtgcaaacaaaagtgtgcatggtctttgtcaattgatacctatgtgcacgtgtgcagaaactgttgttccagctggggtgtctgattaggagggcagatccataaaaggtctaacctaggcaacttcgggaaaggagaccagatcagtagctggaggcactctccagtaggcggtgaggggtttactgagtaggcatgctgaagcccggatattcacccatctcaaaccccccgggctgcaggacaggcacaggccatccctgaggagaaggggagcccttttgggataccacctgaggttatgttcagtgtgctctggtcaagtcccttgctcggggctctgtttggggagagtggtttcattccaaggtactcattattagtatgctgttttgttaactatactccattaaaaagttaaaaaaaaaaagaattaagccttgacactgtatggctgacaggaggctgtgcccagactgagcctggagatttgcgcccgcacatggtcattggttttccgaaaagagagggtaaatttatatagaaatttacaggtatttgggtagtcatttagaccgagggagaccagtgtttccatttctctgcgccccctctgtgaggggaagttcgatacacttgacacctttataaacggagccagataggaagggagtgacttaattcaccttagaacatttcatttggtgtttatttctgaaggtgcaagagctctgtgtaggtttcatttgtgcccgagcatttctggagcactgtgttttctagcagaaactccgagagccagttctcacaatgaaactttaaaacctgtgtaaattgacagagagcagaaggcgatccaagaggcccactcaagtgagtggtggcacgaggcacatgcggtggccctttctgttgtgctggcccatgagagatgggagctattttgtcctcttcgtccattaaaacaaacccctccagaatacctatagtaatataatgaaagccatatctctgtgatctataccgtcaggtatagatcattaaaggacccatggtactgtcaggcactgtggaaccgtgaggcagcggaaaggcaagggcacatttgtacatgttcctctagcttccgccagccgtgacctatgaactcacataggccggttgctcctagtctgacgggctgccctgggaggaaaagctgcaagatgctcagcagagagcaaaggagaggatagtcttggaaaaggccaaggttggggatgccatacaggattacaccaaagggctgtactgagaatgtgggagcattccattccaggtttgtattttcctcagcaagaaaaaagagcagatagaagggcagaggaggatagagaggaagagaaaggagagggagaagagagcagagaagagagagagagagagagagagagagaatctttatactttttggcaagtcctcgaaggtctcaaaatgaaagtgtctatgcaagtgcaaatttttacagttatttatactaattattattattgttattaattattattattactagtctgttgtctcaagaatatgtgcagatttcagagcattaaagagtatttggtttcttttaaagtagttgggtgagccaaggacaccttaaaataattgtcactgttcatctgctatcgcctttctcatggtattttaagttttagaaaagaaacattcttgttctaaaacatatccctctccatagatgacaaaaaaaaatggtgttagcaaaccgaaacctcccccgattcctgtctgacatccgatccatttctcaactgcttgatgatttccgagcgctttttgcatatgttgtcaaaatattcatattattttggtgagggaatggagactcagaaactcagaggacaaacataagcttcaccgaagtctgtctgccagatacaaactaacatacaaacaagacagccgggaaggaaatgtgctggtagcgtgtctgtggagcagggtgggggttagaacagaaggagacctgggcagtgcacgcagaagagatgttacatcatgtgcttctgctcctggcttctgctgactcccaactttgcgctcagcctcatttagaaaacgcttcaaacactgctcttcagggttctgtcagaactcacacacacgtgctcacaccagccccgcttgtgacgtttttatgtacttctatataaatatatacataatatatgttataaacacttgatttatacatatacaaatgcacacatgtagtgtgtttgtgtgtttatgtataaacatataggctcatggtaatagaataattataagtagggtgcaatatgaataatttgcttaatatttgctaagtaaccaaaactttccaacgtcatgtggcagttcatatttccactctcagtgtgggtaaggatgggctacaccacactttcagctctgtgcagcccttggatggaagatgtgttgaaaaaaaaatcacatcttccctgaaacaactgactgaaagccatcctctacattgaatctgttctctggctctttgcaaaggagaaatgcagacaaatggtctccttgtgtcccagtcctgggaaggagaagtgggttttctcttcttgcacatttgggccgtgctcacctttcctggctctatgccctttacactgggctcagagatgaagcagtctagacccaagctgcagggctgtagggaggcaaatgtcttcgaggctgatagcaaagcatccaaaaatctatagcaagatgcgcagcttgaagtcactcctcatccacacggcaagcaagagccagggcatgcagtgctgtccatctctaggactgggcagtggggtccccggtcaagggcagtctttccctaagcctctccttttgcaaatggcactgccagcagtacctggcattaagtcacgaaaaatttctaaaatggcagcacagacccgtgtgccctcattgctctgcccccacatgcctcatcattagagggctccagttttcaaacttgactttccatttggccctgtatcgtggttaaaggaaatctcaacagagggatggccaattgacctaaatccccagatgtccaagtttgcagtgaaagccagttcttcccaaatgtataactggaatgtagggactcaggttgtgatacttcatacaggaatctcagatgttattgtaaagaactgggttgggagggattcatcactaagccaacaataatgcaggagggcgtggctgatcgttaagccaatagtagtgcaggagggcgtggctgctgtgagggctggaatccatctctgctgctaaagttcagggttctcaactcttttcagctgttgcagcccttcacttctttcccttcggcgttatttatttgtgtatttatttatttatttatttatttatctatctatctatcaacttttggtccattcatcaccaacataaagcaaaaacaattttttacatatatgtaaatgtgttgcaagtgaaacactgtgaatctcacaaccacctcctagcaactatgctgccatcttgacgtgcgtctcaggagtcgagacgggaaaagacgaggacgtcattttgcagcctacgcattctgggccaggtccgtgttcgttttatttctttagtctgtgagttaagaaaacaatccgagtggagggtgacggatgttcggcaagttcggtgaagcagcacgagctctttgcagctataggttcgagcaagaagaaaaaccatgggagatggagaagggaaatttgatggaggggtggggtggggtgggggctctgtcttacagctcgtgtagcttactgttgcttaaaaatgtatacaacagctggaaatgttttcaacacaaggtatttgaaataaatgtgaatcttaaatatgtactcccttaaggaatgaacatattatggtgaaatattgctcccccgcgtcccctacaaatctgcctagagatgtggatacctacatttgcttaagcatcagaccagtgtttgtatatacccgggccatacacactcatctcgacgtctctctgcggatgtatttccccttcactggtgacctggtatttagaactccgtcttttcagttggtttatttccctttaatgtgatgtctctgtgccgattattaccggttcttacttgtttttgcaatccgttttgaggtccagtgttttactgagactcattgcatcttggctgatttcaaagtgacacccgaatacagtgtttaaaaaaaaagtttgtttgtaaatcatgtgaccagcttctctcaccctgacatggaatgtctcttgtactacagtgtatttaataataaaagaaaaaaatgatgtcttacaataaataacatcttccacaagagg

SEQ ID NO: 7 - DNA, 4750 bp, Rattus norvegicus
  source 1..4750: mol_type = other DNA
tgtgcgtgcgtgcgtgtgtgtgtgtgtgtgtgtgtgtgtgtgtgtgtgtgtgtgtgtgtgtgagcgtgtgtgtttttggatttcatactaattttctggagtttctgcccctgctctgcgtcagccctcacgtcacttcgccagcagtagcagaggcggcggcggccgccggttagagcccagtcgctgcttcagctgctgttgctgcttctgcggcgctctgctccctgcgctggctacgggaggccgggggagccgcgccgacagtcctctgtggccagggccggcactgtcctgctaccgcagttgctccccagccctgaggtgcgcaccgatatcgatatccgtgccggtttagcggttctgcgacccaaagagtccagggagagccaccgagtggcgcctggcgtataggaccatgcagccgccttgtggcttggagcagcggcccgtgatgttccagccactgtgaaccatttggtcagcgccaacctgctcagccccagcaccgacaggctcagcctctggtacgctcctctcggcgggaggccatcagcaccaagcagcaagagggctcagggaaggcctcccccctccggcgggggacgcctggctcagcgtagggacacgcactctgactgactggcactggcagctcgggatgtcgccctggccgaggtggcatggacccgccatggcgcggctctggggcttatgcttgctggtcttgggcttctggagggcttctcttgcctgccccatgtcctgcaaatgcagcaccactaggatttggtgtaccgagccttctcctggcatcgtggcatttccgaggttggaacctaacagcattgacccagagaacatcaccgaaattctcattgcaaaccagaaaaggttagaaatcatcaatgaagatgatgtcgaagcttacgtggggctgaaaaaccttacaattgtggattccggcttaaagtttgtggcttacaaggcgtttctgaagaacggcaacctgcggcacatcaatttcactcgaaacaagctgacgagtttgtccaggagacatttccgccaccttgacttgtctgacctgatcctgacgggtaatccgttcacgtgttcctgtgacatcatgtggctcaagactctccaggagacgaaatccagccccgacactcaggatttgtattgcctcaatgagagcagcaagaatacccctctggcgaacctgcagattcccaattgtggtctgccgtctgcacgtctggccgctcctaacctcacggtggaggaagggaagtctgtgaccatttcctgcagcgtcgggggtgacccgctccccaccttgtactgggacgttgggaatttggtttccaaacacatgaatgaaacaagccacacacagggctccttaaggataacaaacatttcatcggatgacagtgggaaacaaatctcttgtgtggcagaaaacctcgttggagaagatcaagactctgtgaacctcactgtgcattttgcaccaaccatcacatttctcgaatctccaacctcagaccaccactggtgcatcccattcactgtgagaggcaaccccaagccagcacttcagtggttctacaacggagccatactgaatgaatccaagtacatctgtaccaaaatacacgtcaccaatcacacggagtaccacggctgcctccagctggataaccccactcatatgaataatggagactacaccctaatggccaagaatgaatatgggaaggacgagagacagatttctgctcacttcatgggccggcctggagttgactatgagacaaacccaaattaccctgaagtcctctatgaagactggaccacgccaactgacatcggggatactacaaacaaaagtaatgagatcccctccacggatgttgctgaccaaaccaatcgggagcatctctcggtctatgccgtggtggtgattgcctctgtggtaggattctgcctgctggtgatgctgcttctgctcaagttggcgagacattccaagtttggcatgaaaggcccagcttccgtcatcagcaacgacgatgactctgccagccctctccaccacatctccaacgggagcaacactccgtcttcttcggagggcgggcccgatgctgtcatcattgggatgaccaagatccctgtcattgaaaacccccagtacttcggtatcaccaacagccagctcaagccggacacatttgttcagcacatcaagagacacaacatcgttctgaagagggagcttggagaaggagcctttgggaaagttttcctagcggagtgctataacctctgccccgagcaggataagatcctggtggccgtgaagacgctgaaggacgccagcgacaatgctcgcaaggactttcatcgcgaagccgagctgctgaccaacctccagcacgagcacattgtcaagttctacggtgtctgtgtggagggcgacccactcatcatggtctttgagtacatgaagcacggggacctcaacaagttccttagggcacacgggccagatgcagtgctgatggcagagggtaacccgcccaccgagctgacgcagtcgcagatgctgcacatcgctcagcaaatcgcagcaggcatggtctacctggcatcccaacacttcgtgcaccgagacctggccacccggaactgcttggtaggagagaacctgctggtgaaaattggggacttcgggatgtcccgggatgtatacagcaccgactactaccgggttggtggccacacaatgttgcccatccgatggatgcctccagagagcatcatgtacaggaaattcaccaccgagagtgacgtctggagcctgggagttgtgttgtgggagatcttcacctacggcaagcagccctggtatcagctatcaaacaacgaggtgatagaatgcatcacccagggcagagtccttcagcggcctcgcacgtgtccccaggaggtgtacgagctgatgctgggatgctggcagcgggaaccacacacaaggaagaacatcaagaacatccacacactccttcagaacttggcgaaggcgtcgcccgtctacctggacatcctaggctagactccctcttctcccagacggcccttcccaaggcacccctcagacctcttaactgccgctgatgtcaccaccttgctgtccttcgctctgacagtgttaacaagacaaggagcggctctccggggtgaggcagtgcgcacttccccatccacagacagtatcgactcgcttctggctttgtcgctttctctccctttggtttgtttctttcttttgcccattctccatttatttatttatttatttatttatttatttatttatttatctatctatctatctatctatctatctatttatttatttattggtcttcactgcttcatggtcctcggcctctctccttgaccgatctggcttctgtactcctattcactgtacatagacaaaggccttaacaaacctgatttgttatatcagcagacactccagtttgcccaccacaactaacaatgccttgttgtattcctgcctttgatgtggatgaaaaaaagggaaaaaaaaataatcaaacatctgacttaaaccgtcacttccgatgtacagacacggggcgtttctatggattcacttctatctatctatttatttatttatctatttatttatttctcttctttgttgttttccggtggttttagcctgtgtatgagaagggaaagtcatgtacagtctgggaaaactttatctgtgggaaatggaaaccagaaagggaaagaagctttaccataaagcacagcaggagtgagacacagaaaagccattggatcagccagagtccgtcctgcataggaaaacccagcagccatcaggctggaggatcatgttcggcactgacccccgaggacctttctgaggaggacacagaatgttaaactctgcatcatggacacagtttccgatcacagatactggccttcaatggaaaaaaaaaaaaacccagatagttcttgtgagacctggacagcacgtccaacatccagacattgtggtcgggcacagtgacagagttgatgcatttctcacgggttattctacagagcttttgtcaagtccaatggaaggaggtagattcttgttcagatatgatttcgggaaaaaccgagtccttgacaaagacaggagacaccctcagttgggaggcaagtttctcttaccttggactttctcacacagcaattctcacccccaccccctccactctcacctgtcttgtaactgtgcaaacaaaagtgtgcatggtctttgtcagttgatacctttgtgcacctctgtgcagaaactgctgtctgtcccggctgtggtacccgatcagtggggtagatccacgaaaggtctcattttaggccgctttgggaaggtaaccagatcggtagctggaagcactctccagtaggtggcgaagggtgagtgggtctgctgaagcctgcatatcttcacccacctcaaacccaccgggctgcacaggggacaggcacaggccacccctgagggacagggaagctctcttgggataccacctgagtttacattcagtgtgctcaggtcaagtctctcgctcggggctctgtttcggggagaatggtttcattccaacgcactcattatcaggattctgttttc

SEQ ID NO: 8 - DNA, 4057 bp, Homo sapiens
  source 1..4057: mol_type = other DNA
gggagcaggagcctcgctggctgcttcgctcgcgctctacgcgctcagtccccggcggtagcaggagcctggacccaggcgccggcggcgggcgtgaggcgccggagcccggcctcgaggtgcataccggacccccattcgcatctaacaaggaatctgcgccccagagagtcccggacgccgccggtcggtgcccggcgcgccgggccatgcagcgacggccgccgcggagctccgagcagcggtagcgcccccctgtaaagcggttcgctatgccgggaccactgtgaaccctgccgcctgccggaacactcttcgctccggaccagctcagcctctgataagctggactcggcacgcccgcaacaagcaccgaggagttaagagagccgcaagcgcagggaaggcctccccgcacgggtgggggaaagcggccggtgcagcgcggggacaggcactcgggctggcactggctgctagggatgtcgtcctggataaggtggcatggacccgccatggcgcggctctggggcttctgctggctggttgtgggcttctggagggccgctttcgcctgtcccacgtcctgcaaatgcagtgcctctcggatctggtgcagcgacccttctcctggcatcgtggcatttccgagattggagcctaacagtgtagatcctgagaacatcaccgaaattttcatcgcaaaccagaaaaggttagaaatcatcaacgaagatgatgttgaagcttatgtgggactgagaaatctgacaattgtggattctggattaaaatttgtggctcataaagcatttctgaaaaacagcaacctgcagcacatcaattttacccgaaacaaactgacgagtttgtctaggaaacatttccgtcaccttgacttgtctgaactgatcctggtgggcaatccatttacatgctcctgtgacattatgtggatcaagactctccaagaggctaaatccagtccagacactcaggatttgtactgcctgaatgaaagcagcaagaatattcccctggcaaacctgcagatacccaattgtggtttgccatctgcaaatctggccgcacctaacctcactgtggaggaaggaaagtctatcacattatcctgtagtgtggcaggtgatccggttcctaatatgtattgggatgttggtaacctggtttccaaacatatgaatgaaacaagccacacacagggctccttaaggataactaacatttcatccgatgacagtgggaagcagatctcttgtgtggcggaaaatcttgtaggagaagatcaagattctgtcaacctcactgtgcattttgcaccaactatcacatttctcgaatctccaacctcagaccaccactggtgcattccattcactgtgaaaggcaaccccaaaccagcgcttcagtggttctataacggggcaatattgaatgagtccaaatacatctgtactaaaatacatgttaccaatcacacggagtaccacggctgcctccagctggataatcccactcacatgaacaatggggactacactctaatagccaagaatgagtatgggaaggatgagaaacagatttctgctcacttcatgggctggcctggaattgacgatggtgcaaacccaaattatcctgatgtaatttatgaagattatggaactgcagcgaatgacatcggggacaccacgaacagaagtaatgaaatcccttccacagacgtcactgataaaaccggtcgggaacatctctcggtctatgctgtggtggtgattgcgtctgtggtgggattttgccttttggtaatgctgtttctgcttaagttggcaagacactccaagtttggcatgaaagatttctcatggtttggatttgggaaagtaaaatcaagacaaggtgttggcccagcctccgttatcagcaatgatgatgactctgccagcccactccatcacatctccaatgggagtaacactccatcttcttcggaaggtggcccagatgctgtcattattggaatgaccaagatccctgtcattgaaaatccccagtactttggcatcaccaacagtcagctcaagccagacacatttgttcagcacatcaagcgacataacattgttctgaaaagggagctaggcgaaggagcctttggaaaagtgttcctagctgaatgctataacctctgtcctgagcaggacaagatcttggtggcagtgaagaccctgaaggatgccagtgacaatgcacgcaaggacttccaccgtgaggccgagctcctgaccaacctccagcatgagcacatcgtcaagttctatggcgtctgcgtggagggcgaccccctcatcatggtctttgagtacatgaagcatggggacctcaacaagttcctcagggcacacggccctgatgccgtgctgatggctgagggcaacccgcccacggaactgacgcagtcgcagatgctgcatatagcccagcagatcgccgcgggcatggtctacctggcgtcccagcacttcgtgcaccgcgatttggccaccaggaactgcctggtcggggagaacttgctggtgaaaatcggggactttgggatgtcccgggacgtgtacagcactgactactacagggtcggtggccacacaatgctgcccattcgctggatgcctccagagagcatcatgtacaggaaattcacgacggaaagcgacgtctggagcctgggggtcgtgttgtgggagattttcacctatggcaaacagccctggtaccagctgtcaaacaatgaggtgatagagtgtatcactcagggccgagtcctgcagcgaccccgcacgtgcccccaggaggtgtatgagctgatgctggggtgctggcagcgagagccccacatgaggaagaacatcaagggcatccataccctccttcagaacttggccaaggcatctccggtctacctggacattctaggctagggcccttttccccagaccgatccttcccaacgtactcctcagacgggctgagaggatgaacatcttttaactgccgctggaggccaccaagctgctctccttcactctgacagtattaacatcaaagactccgagaagctctcgagggaagcagtgtgtacttcttcatccatagacacagtattgacttctttttggcattatctctttctctctttccatctcccttggttgttcctttttctttttttaaattttctttttcttcttttttttcgtcttccctgcttcacgattcttaccctttcttttgaatcaatctggcttctgcattactattaactctgcatagacaaaggccttaacaaacgtaatttgttatatcagcagacactccagtttgcccaccacaactaacaatgccttgttgtattcctgcctttgatgtggatgaaaaaaagggaaaacaaatatttcacttaaactttgtcacttctgctgtacagatatcgagagtttctatggattcacttctatttatttattattattactgttcttattgtttttggatggcttaagcctgtgtataaaaaagaaaacttgtgttcaatctgtgaagcctttatctatgggagattaaaaccagagagaaagaagatttattatgaaccgcaatatgggaggaacaaagacaaccactgggatcagctggtgtcagtccctacttaggaaatactcagcaactgttagctgggaagaatgtattcggcaccttcccctgaggacctttctgaggagtaaaaagactactggcctctgtgccatggatgattcttttcccatcaccagaaatgatagcgtgcagtagagagcaaagatggcttccgtgagacacaagatggcgcatagtgtgctcggacacagttttgtcttcgtaggttgtgatgatagcactggtttgtttctcaagcgctatccacagaacctttgtcaacttcagttgaaaagaggtggattcatgtccagagctcatttcggggtcaggtgggaaagcc

SEQ ID NO: 9 - DNA, 2466 bp, Mus musculus
  misc_feature 1..93: note = Signal Peptide
  misc_feature 94..1287: note = Extracellular Domain
  misc_feature 1288..1359: note = Transmembrane Domain
  misc_feature 1360..2463: note = Cytoplasmic Domain
  source 1..2466: mol_type = other DNA
atgtcgccctggctgaagtggcatggacccgccatggcgcggctctggggcttatgcctgctggtcttgggcttctggagggcctctctcgcctgcccgacgtcctgcaaatgcagttccgctaggatttggtgtactgagccttctccaggcatcgtggcattcccgaggttggaacctaacagcgttgacccggagaacatcacggaaattctcattgcaaaccagaaaaggctagaaatcatcaatgaagatgacgttgaagcttacgtggggctgagaaaccttacaattgtggattccggcttaaagtttgtggcttacaaagcgtttctgaaaaacagcaacctgcggcacataaatttcacacgaaacaagctgacgagtttgtccaggagacatttccgccaccttgacttgtctgacctgatcctgacgggtaatccgttcacgtgctcctgcgacatcatgtggctcaagactctccaggagactaaatccagccccgacactcaggatttgtactgcctcaatgagagcagcaagaacatgcccctggcgaacctgcagatacccaattgtggtctgccatctgcacgtctggctgctcctaacctcaccgtggaggaaggaaagtctgtgaccctttcctgcagtgtggggggtgacccactccccaccttgtactgggacgttgggaatttggtttccaagcacatgaatgaaacaagccacacacagggctccttaaggataacgaacatttcatctgatgacagtggaaagcaaatctcttgtgtggcagaaaaccttgtaggagaagatcaagattctgtgaacctcactgtgcattttgcgccaactatcacgtttctcgagtctccaacctcagatcaccactggtgcattccattcactgtgagaggcaaccccaagcctgcgcttcagtggttctacaatggggccatactgaatgagtccaagtacatctgtactaagatccacgtcaccaatcacacggagtaccatggctgcctccagctggataaccccactcatatgaataacggagactacaccctgatggccaagaacgagtatgggaaggatgagagacagatctccgctcacttcatgggccggcctggagtcgactacgagacaaacccaaattaccctgaagtcctctatgaagactggaccacgccaactgacattggggatactacgaacaaaagtaatgaaatcccctccacggatgttgctgaccaaagcaatcgggagcatctctcggtctatgccgtggtggtgattgcatctgtggtgggattctgcctgctggtgatgttgctcctgctcaagttggcgagacattccaagtttggcatgaaaggcccagcttcggtcatcagcaacgacgatgactctgccagccccctccaccacatctccaatgggagtaacactccatcttcttcggagggcggtcccgacgctgtcattattggaatgaccaagattcctgttattgaaaacccccagtactttggcatcaccaacagtcagctcaagccagacacatttgttcagcatatcaagagacacaacatcgttctgaagagggaacttggggaaggagccttcgggaaagttttccttgccgagtgctacaacctctgcccagagcaggataagatcctggtggctgtgaagacgctgaaggacgccagcgacaatgcacgcaaggactttcatcgggaagctgagctgctgaccaacctccagcacgagcacattgtcaagttctacggtgtctgtgtggagggcgacccactcatcatggtctttgagtacatgaagcacggggacctcaacaagttccttagggcacacgggcccgacgcagtgctgatggcagagggtaacccgcccacagagctgacgcagtcgcagatgctgcacatcgctcagcaaatcgcagcaggtatggtctacctggcgtcccaacactttgtgcaccgtgacctggccacccggaactgcctggtgggagagaacctgctggtgaaaattggggactttgggatgtcccgagatgtgtacagcaccgactactatcgggtcggtggccacacaatgttgcccatccgatggatgcctccagagagcatcatgtacaggaaattcaccaccgagagcgacgtctggagcctgggcgttgtgttgtgggagatcttcacctacggcaagcagccctggtatcagctatcgaacaatgaggtgatagagtgcatcacccagggaagagtccttcagcggcctcgaacgtgtccccaggaggtgtatgagctcatgcttggatgctggcagcgggaaccacacacccggaagaacatcaagagcatccacaccctccttcagaacttggccaaggcatctcccgtctacctggatatcctaggctag

SEQ ID NO: 10 - DNA, 2466 bp, Rattus norvegicus
  misc_feature 1..93: note = Signal Peptide
  misc_feature 94..1287: note = Extracellular Domain
  misc_feature 1288..1359: note = Transmembrane Domain
  misc_feature 1360..2463: note = Cytoplasmic Domain
  source 1..2466: mol_type = other DNA
atgtcgccctggccgaggtggcatggacccgccatggcgcggctctggggcttatgcttgctggtcttgggcttctggagggcttctcttgcctgccccatgtcctgcaaatgcagcaccactaggatttggtgtaccgagccttctcctggcatcgtggcatttccgaggttggaacctaacagcattgacccagagaacatcaccgaaattctcattgcaaaccagaaaaggttagaaatcatcaatgaagatgatgtcgaagcttacgtggggctgaaaaaccttacaattgtggattccggcttaaagtttgtggcttacaaggcgtttctgaagaacggcaacctgcggcacatcaatttcactcgaaacaagctgacgagtttgtccaggagacatttccgccaccttgacttgtctgacctgatcctgacgggtaatccgttcacgtgttcctgtgacatcatgtggctcaagactctccaggagacgaaatccagccccgacactcaggatttgtattgcctcaatgagagcagcaagaatacccctctggcgaacctgcagattcccaattgtggtctgccgtctgcacgtctggccgctcctaacctcacggtggaggaagggaagtctgtgaccatttcctgcagcgtcgggggtgacccgctccccaccttgtactgggacgttgggaatttggtttccaaacacatgaatgaaacaagccacacacagggctccttaaggataacaaacatttcatcggatgacagtgggaaacaaatctcttgtgtggcagaaaacctcgttggagaagatcaagactctgtgaacctcactgtgcattttgcaccaaccatcacatttctcgaatctccaacctcagaccaccactggtgcatcccattcactgtgagaggcaaccccaagccagcacttcagtggttctacaacggagccatactgaatgaatccaagtacatctgtaccaaaatacacgtcaccaatcacacggagtaccacggctgcctccagctggataaccccactcatatgaataatggagactacaccctaatggccaagaatgaatatgggaaggacgagagacagatttctgctcacttcatgggccggcctggagttgactatgagacaaacccaaattaccctgaagtcctctatgaagactggaccacgccaactgacatcggggatactacaaacaaaagtaatgagatcccctccacggatgttgctgaccaaaccaatcgggagcatctctcggtctatgccgtggtggtgattgcctctgtggtaggattctgcctgctggtgatgctgcttctgctcaagttggcgagacattccaagtttggcatgaaaggcccagcttccgtcatcagcaacgacgatgactctgccagccctctccaccacatctccaacgggagcaacactccgtcttcttcggagggcgggcccgatgctgtcatcattgggatgaccaagatccctgtcattgaaaacccccagtacttcggtatcaccaacagccagctcaagccggacacatttgttcagcacatcaagagacacaacatcgttctgaagagggagcttggagaaggagcctttgggaaagttttcctagcggagtgctataacctctgccccgagcaggataagatcctggtggccgtgaagacgctgaaggacgccagcgacaatgctcgcaaggactttcatcgcgaagccgagctgctgaccaacctccagcacgagcacattgtcaagttctacggtgtctgtgtggagggcgacccactcatcatggtctttgagtacatgaagcacggggacctcaacaagttccttagggcacacgggccagatgcagtgctgatggcagagggtaacccgcccaccgagctgacgcagtcgcagatgctgcacatcgctcagcaaatcgcagcaggcatggtctacctggcatcccaacacttcgtgcaccgagacctggccacccggaactgcttggtaggagagaacctgctggtgaaaattggggacttcgggatgtcccgggatgtatacagcaccgactactaccgggttggtggccacacaatgttgcccatccgatggatgcctccagagagcatcatgtacaggaaattcaccaccgagagtgacgtctggagcctgggagttgtgttgtgggagatcttcacctacggcaagcagccctggtatcagctatcaaacaacgaggtgatagaatgcatcacccagggcagagtccttcagcggcctcgcacgtgtccccaggaggtgtacgagctgatgctgggatgctggcagcgggaaccacacacaaggaagaacatcaagaacatccacacactccttcagaacttggcgaaggcgtcgcccgtctacctggacatcctaggctag

SEQ ID NO: 11 - DNA, 2517 bp, Homo sapiens
  misc_feature 1..93: note = Signal Peptide
  misc_feature 94..1290: note = Extracellular Domain
  misc_feature 1291..1362: note = Transmembrane Domain
  misc_feature 1363..2514: note = Cytoplasmic Domain
  source 1..2517: mol_type = other DNA
atgtcgtcctggataaggtggcatggacccgccatggcgcggctctggggcttctgctggctggttgtgggcttctggagggccgctttcgcctgtcccacgtcctgcaaatgcagtgcctctcggatctggtgcagcgacccttctcctggcatcgtggcatttccgagattggagcctaacagtgtagatcctgagaacatcaccgaaattttcatcgcaaaccagaaaaggttagaaatcatcaacgaagatgatgttgaagcttatgtgggactgagaaatctgacaattgtggattctggattaaaatttgtggctcataaagcatttctgaaaaacagcaacctgcagcacatcaattttacccgaaacaaactgacgagtttgtctaggaaacatttccgtcaccttgacttgtctgaactgatcctggtgggcaatccatttacatgctcctgtgacattatgtggatcaagactctccaagaggctaaatccagtccagacactcaggatttgtactgcctgaatgaaagcagcaagaatattcccctggcaaacctgcagatacccaattgtggtttgccatctgcaaatctggccgcacctaacctcactgtggaggaaggaaagtctatcacattatcctgtagtgtggcaggtgatccggttcctaatatgtattgggatgttggtaacctggtttccaaacatatgaatgaaacaagccacacacagggctccttaaggataactaacatttcatccgatgacagtgggaagcagatctcttgtgtggcggaaaatcttgtaggagaagatcaagattctgtcaacctcactgtgcattttgcaccaactatcacatttctcgaatctccaacctcagaccaccactggtgcattccattcactgtgaaaggcaaccccaaaccagcgcttcagtggttctataacggggcaatattgaatgagtccaaatacatctgtactaaaatacatgttaccaatcacacggagtaccacggctgcctccagctggataatcccactcacatgaacaatggggactacactctaatagccaagaatgagtatgggaaggatgagaaacagatttctgctcacttcatgggctggcctggaattgacgatggtgcaaacccaaattatcctgatgtaatttatgaagattatggaactgcagcgaatgacatcggggacaccacgaacagaagtaatgaaatcccttccacagacgtcactgataaaaccggtcgggaacatctctcggtctatgctgtggtggtgattgcgtctgtggtgggattttgccttttggtaatgctgtttctgcttaagttggcaagacactccaagtttggcatgaaagatttctcatggtttggatttgggaaagtaaaatcaagacaaggtgttggcccagcctccgttatcagcaatgatgatgactctgccagcccactccatcacatctccaatgggagtaacactccatcttcttcggaaggtggcccagatgctgtcattattggaatgaccaagatccctgtcattgaaaatccccagtactttggcatcaccaacagtcagctcaagccagacacatttgttcagcacatcaagcgacataacattgttctgaaaagggagctaggcgaaggagcctttggaaaagtgttcctagctgaatgctataacctctgtcctgagcaggacaagatcttggtggcagtgaagaccctgaaggatgccagtgacaatgcacgcaaggacttccaccgtgaggccgagctcctgaccaacctccagcatgagcacatcgtcaagttctatggcgtctgcgtggagggcgaccccctcatcatggtctttgagtacatgaagcatggggacctcaacaagttcctcagggcacacggccctgatgccgtgctgatggctgagggcaacccgcccacggaactgacgcagtcgcagatgctgcatatagcccagcagatcgccgcgggcatggtctacctggcgtcccagcacttcgtgcaccgcgatttggccaccaggaactgcctggtcggggagaacttgctggtgaaaatcggggactttgggatgtcccgggacgtgtacagcactgactactacagggtcggtggccacacaatgctgcccattcgctggatgcctccagagagcatcatgtacaggaaattcacgacggaaagcgacgtctggagcctgggggtcgtgttgtgggagattttcacctatggcaaacagccctggtaccagctgtcaaacaatgaggtgatagagtgtatcactcagggccgagtcctgcagcgaccccgcacgtgcccccaggaggtgtatgagctgatgctggggtgctggcagcgagagccccacatgaggaagaacatcaagggcatccataccctccttcagaacttggccaaggcatctccggtctacctggacattctaggctag

SEQ ID NO: 12 - DNA, 2469 bp, synthetic construct
  misc_feature 1..2469: note = Synthetic
  misc_feature 1..93: note = Signal Peptide
  misc_feature 1..93: note = Mouse Sequence
  misc_feature 94..1290: note = Extracellular Domain
  misc_feature 94..1296: note = Human Sequence
  misc_feature 1291..1362: note = Transmembrane Domain
  misc_feature 1297..2466: note = Mouse Sequence
  misc_feature 1363..2466: note = Cytoplasmic Domain
  source 1..2469: mol_type = other DNA
atgtcgccctggctgaagtggcatggacccgccatggcgcggctctggggcttatgcctgctggtcttgggcttctggagggcctctctcgcctgtcccacgtcctgcaaatgcagtgcctctcggatctggtgcagcgacccttctcctggcatcgtggcatttccgagattggagcctaacagtgtagatcctgagaacatcaccgaaattttcatcgcaaaccagaaaaggttagaaatcatcaacgaagatgatgttgaagcttatgtgggactgagaaatctgacaattgtggattctggattaaaatttgtggctcataaagcatttctgaaaaacagcaacctgcagcacatcaattttacccgaaacaaactgacgagtttgtctaggaaacatttccgtcaccttgacttgtctgaactgatcctggtgggcaatccatttacatgctcctgtgacattatgtggatcaagactctccaagaggctaaatccagtccagacactcaggatttgtactgcctgaatgaaagcagcaagaatattcccctggcaaacctgcagatacccaattgtggtttgccatctgcaaatctggccgcacctaacctcactgtggaggaaggaaagtctatcacattatcctgtagtgtggcaggtgatccggttcctaatatgtattgggatgttggtaacctggtttccaaacatatgaatgaaacaagccacacacagggctccttaaggataactaacatttcatccgatgacagtgggaagcagatctcttgtgtggcggaaaatcttgtaggagaagatcaagattctgtcaacctcactgtgcattttgcaccaactatcacatttctcgaatctccaacctcagaccaccactggtgcattccattcactgtgaaaggcaaccccaaaccagcgcttcagtggttctataacggggcaatattgaatgagtccaaatacatctgtactaaaatacatgttaccaatcacacggagtaccacggctgcctccagctggataatcccactcacatgaacaatggggactacactctaatagccaagaatgagtatgggaaggatgagaaacagatttctgctcacttcatgggctggcctggaattgacgatggtgcaaacccaaattatcctgatgtaatttatgaagattatggaactgcagcgaatgacatcggggacaccacgaacagaagtaatgaaatcccttccacagacgtcactgataaaaccggtcgggaacatctctcggtctatgccgtggtggtgattgcatctgtggtgggattctgcctgctggtgatgttgctcctgctcaagttggcgagacattccaagtttggcatgaaaggcccagcttcggtcatcagcaacgacgatgactctgccagccccctccaccacatctccaatgggagtaacactccatcttcttcggagggcggtcccgacgctgtcattattggaatgaccaagattcctgttattgaaaacccccagtactttggcatcaccaacagtcagctcaagccagacacatttgttcagcatatcaagagacacaacatcgttctgaagagggaacttggggaaggagccttcgggaaagttttccttgccgagtgctacaacctctgcccagagcaggataagatcctggtggctgtgaagacgctgaaggacgccagcgacaatgcacgcaaggactttcatcgggaagctgagctgctgaccaacctccagcacgagcacattgtcaagttctacggtgtctgtgtggagggcgacccactcatcatggtctttgagtacatgaagcacggggacctcaacaagttccttagggcacacgggcccgacgcagtgctgatggcagagggtaacccgcccacagagctgacgcagtcgcagatgctgcacatcgctcagcaaatcgcagcaggtatggtctacctggcgtcccaacactttgtgcaccgtgacctggccacccggaactgcctggtgggagagaacctgctggtgaaaattggggactttgggatgtcccgagatgtgtacagcaccgactactatcgggtcggtggccacacaatgttgcccatccgatggatgcctccagagagcatcatgtacaggaaattcaccaccgagagcgacgtctggagcctgggcgttgtgttgtgggagatcttcacctacggcaagcagccctggtatcagctatcgaacaatgaggtgatagagtgcatcacccagggaagagtccttcagcggcctcgaacgtgtccccaggaggtgtatgagctcatgcttggatgctggcagcgggaaccacacacccggaagaacatcaagagcatccacaccctccttcagaacttggccaaggcatctcccgtctacctggatatcctaggctag

SEQ ID NO: 13 - DNA, 2469 bp, synthetic construct
  misc_feature 1..2469: note = Synthetic
  misc_feature 1..93: note = Signal Peptide
  misc_feature 1..93: note = Rat Sequence
  misc_feature 94..1290: note = Extracellular Domain
  misc_feature 94..1296: note = Human Sequence
  misc_feature 1291..1362: note = Transmembrane Domain
  misc_feature 1297..2466: note = Rat Sequence
  misc_feature 1363..2466: note = Cytoplasmic Domain
  source 1..2469: mol_type = other DNA
atgtcgccctggccgaggtggcatggacccgccatggcgcggctctggggcttatgcttgctggtcttgggcttctggagggcttctcttgcctgtcccacgtcctgcaaatgcagtgcctctcggatctggtgcagcgacccttctcctggcatcgtggcatttccgagattggagcctaacagtgtagatcctgagaacatcaccgaaattttcatcgcaaaccagaaaaggttagaaatcatcaacgaagatgatgttgaagcttatgtgggactgagaaatctgacaattgtggattctggattaaaatttgtggctcataaagcatttctgaaaaacagcaacctgcagcacatcaattttacccgaaacaaactgacgagtttgtctaggaaacatttccgtcaccttgacttgtctgaactgatcctggtgggcaatccatttacatgctcctgtgacattatgtggatcaagactctccaagaggctaaatccagtccagacactcaggatttgtactgcctgaatgaaagcagcaagaatattcccctggcaaacctgcagatacccaattgtggtttgccatctgcaaatctggccgcacctaacctcactgtggaggaaggaaagtctatcacattatcctgtagtgtggcaggtgatccggttcctaatatgtattgggatgttggtaacctggtttccaaacatatgaatgaaacaagccacacacagggctccttaaggataactaacatttcatccgatgacagtgggaagcagatctcttgtgtggcggaaaatcttgtaggagaagatcaagattctgtcaacctcactgtgcattttgcaccaactatcacatttctcgaatctccaacctcagaccaccactggtgcattccattcactgtgaaaggcaaccccaaaccagcgcttcagtggttctataacggggcaatattgaatgagtccaaatacatctgtactaaaatacatgttaccaatcacacggagtaccacggctgcctccagctggataatcccactcacatgaacaatggggactacactctaatagccaagaatgagtatgggaaggatgagaaacagatttctgctcacttcatgggctggcctggaattgacgatggtgcaaacccaaattatcctgatgtaatttatgaagattatggaactgcagcgaatgacatcggggacaccacgaacagaagtaatgaaatcccttccacagacgtcactgataaaaccggtcgggaacatctctcggtctatgccgtggtggtgattgcctctgtggtaggattctgcctgctggtgatgctgcttctgctcaagttggcgagacattccaagtttggcatgaaaggcccagcttccgtcatcagcaacgacgatgactctgccagccctctccaccacatctccaacgggagcaacactccgtcttcttcggagggcgggcccgatgctgtcatcattgggatgaccaagatccctgtcattgaaaacccccagtacttcggtatcaccaacagccagctcaagccggacacatttgttcagcacatcaagagacacaacatcgttctgaagagggagcttggagaaggagcctttgggaaagttttcctagcggagtgctataacctctgccccgagcaggataagatcctggtggccgtgaagacgctgaaggacgccagcgacaatgctcgcaaggactttcatcgcgaagccgagctgctgaccaacctccagcacgagcacattgtcaagttctacggtgtctgtgtggagggcgacccactcatcatggtctttgagtacatgaagcacggggacctcaacaagttccttagggcacacgggccagatgcagtgctgatggcagagggtaacccgcccaccgagctgacgcagtcgcagatgctgcacatcgctcagcaaatcgcagcaggcatggtctacctggcatcccaacacttcgtgcaccgagacctggccacccggaactgcttggtaggagagaacctgctggtgaaaattggggacttcgggatgtcccgggatgtatacagcaccgactactaccgggttggtggccacacaatgttgcccatccgatggatgcctccagagagcatcatgtacaggaaattcaccaccgagagtgacgtctggagcctgggagttgtgttgtgggagatcttcacctacggcaagcagccctggtatcagctatcaaacaacgaggtgatagaatgcatcacccagggcagagtccttcagcggcctcgcacgtgtccccaggaggtgtacgagctgatgctgggatgctggcagcgggaaccacacacaaggaagaacatcaagaacatccacacactccttcagaacttggcgaaggcgtcgcccgtctacctggacatcctaggctag

SEQ ID NO: 14 - DNA, 22 bp, synthetic construct
  misc_feature 1..22: note = Synthetic
  source 1..22: mol_type = other DNA
aggtgggtaggtcctggaagtg

SEQ ID NO: 15 - DNA, 20 bp, synthetic construct
  misc_feature 1..20: note = Synthetic
  source 1..20: mol_type = other DNA
aatgctgtcccaagagtggg

SEQ ID NO: 16 - DNA, 21 bp, synthetic construct
  misc_feature 1..21: note = Synthetic
  source 1..21: mol_type = other DNA
gtcctgcatcccttgtctttg

SEQ ID NO: 17 - DNA, 21 bp, synthetic construct
  misc_feature 1..21: note = Synthetic
  source 1..21: mol_type = other DNA
atgtgggcgttgtgcagtctc

SEQ ID NO: 18 - DNA, 24 bp, synthetic construct
  misc_feature 1..24: note = Synthetic
  source 1..24: mol_type = other DNA
cgctgcagtgcattgaactcagca

SEQ ID NO: 19 - DNA, 20 bp, synthetic construct
  misc_feature 1..20: note = Synthetic
  source 1..20: mol_type = other DNA
ctgtggagggacgtgaccag

SEQ ID NO: 20 - DNA, 22 bp, synthetic construct
  misc_feature 1..22: note = Synthetic
  source 1..22: mol_type = other DNA
tccgctaggatttggtgtactg

SEQ ID NO: 21 - DNA, 24 bp, synthetic construct
  misc_feature 1..24: note = Synthetic
  source 1..24: mol_type = other DNA
agccttctccaggcatcgtggcat

SEQ ID NO: 22 - DNA, 19 bp, synthetic construct
  misc_feature 1..19: note = Synthetic
  source 1..19: mol_type = other DNA
tccgggtcaacgctgttag

SEQ ID NO: 23 - DNA, 18 bp, synthetic construct
  misc_feature 1..18: note = Synthetic
  source 1..18: mol_type = other DNA
tcctgcgagggttctgac

SEQ ID NO: 24 - DNA, 29 bp, synthetic construct
  misc_feature 1..29: note = Synthetic
  source 1..29: mol_type = other DNA
tgggtgctcatatgccagagaaattgtca

SEQ ID NO: 25 - DNA, 22 bp, synthetic construct
  misc_feature 1..22: note = Synthetic
  source 1..22: mol_type = other DNA
cgatctgtgatggcctgcttac

SEQ ID NO: 26 - DNA, 22 bp, synthetic construct
  misc_feature 1..22: note = Synthetic
  source 1..22: mol_type = other DNA
gggctcaggcaggtatatgttg

SEQ ID NO: 27 - DNA, 27 bp, synthetic construct
  misc_feature 1..27: note = Synthetic
  source 1..27: mol_type = other DNA
acagatgctgtcccaaacatagcaaga

SEQ ID NO: 28 - DNA, 23 bp, synthetic construct
  misc_feature 1..23: note = Synthetic
  source 1..23: mol_type = other DNA
ccaaccctaagccagtgaaacag

SEQ ID NO: 29 - DNA, 20 bp, synthetic construct
  misc_feature 1..20: note = Synthetic
  source 1..20: mol_type = other DNA
gtgctggagaccaggagact

SEQ ID NO: 30 - DNA, 28 bp, synthetic construct
  misc_feature 1..28: note = Synthetic
  source 1..28: mol_type = other DNA
tgccatactcagtttatacggtgctgac

SEQ ID NO: 31 - DNA, 20 bp, synthetic construct
  misc_feature 1..20: note = Synthetic
  source 1..20: mol_type = other DNA
gcctggtggctcagtcaatg

SEQ ID NO: 32 - DNA, 19 bp, synthetic construct
  misc_feature 1..19: note = Synthetic
  source 1..19: mol_type = other DNA
gcagacactggatgggtca

SEQ ID NO: 33 - DNA, 26 bp, synthetic construct
  misc_feature 1..26: note = Synthetic
  source 1..26: mol_type = other DNA
ccattcgcgagttatgagaagctgca

SEQ ID NO: 34 - DNA, 22 bp, synthetic construct
  misc_feature 1..22: note = Synthetic
  source 1..22: mol_type = other DNA
acagggttagctggtgaatgga

SEQ ID NO: 35 - DNA, 19 bp, synthetic construct
  misc_feature 1..19: note = Synthetic
  source 1..19: mol_type = other DNA
tcggagcacaggactacag

SEQ ID NO: 36 - DNA, 25 bp, synthetic construct
  misc_feature 1..25: note = Synthetic
  source 1..25: mol_type = other DNA
caagaggaactgtgtccaggaaagc

SEQ ID NO: 37 - DNA, 22 bp, synthetic construct
  misc_feature 1..22: note = Synthetic
  source 1..22: mol_type = other DNA
agcgtgcctcacctaacctcta

SEQ ID NO: 38 - DNA, 19 bp, synthetic construct
  misc_feature 1..19: note = Synthetic
  source 1..19: mol_type = other DNA
gcacagcactgtaaaggca

SEQ ID NO: 39 - DNA, 29 bp, synthetic construct
  misc_feature 1..29: note = Synthetic
  source 1..29: mol_type = other DNA
acggaactcgaaggaattggtattgttgt

SEQ ID NO: 40 - DNA, 23 bp, synthetic construct
  misc_feature 1..23: note = Synthetic
  source 1..23: mol_type = other DNA
acacagctatgggagaaagactg

SEQ ID NO: 41 - DNA, 23 bp, synthetic construct
  misc_feature 1..23: note = Synthetic
  source 1..23: mol_type = other DNA
ccggttggcgagtgcgcatgcac

SEQ ID NO: 42 - DNA, 23 bp, synthetic construct
  misc_feature 1..23: note = Synthetic
  source 1..23: mol_type = other DNA
ccttccggttggcgagtgcgcat

SEQ ID NO: 43 - DNA, 23 bp, synthetic construct
  misc_feature 1..23: note = Synthetic
  source 1..23: mol_type = other DNA
ccaagggtgcgttgatggatcta

SEQ ID NO: 44 - DNA, 23 bp, synthetic construct
  misc_feature 1..23: note = Synthetic
  source 1..23: mol_type = other DNA
gaatgccaagggtgcgttgatgg

SEQ ID NO: 45 - DNA, 23 bp, synthetic construct
  misc_feature 1..23: note = Synthetic
  source 1..23: mol_type = other DNA
ctgggtgattgggactgagaaag

SEQ ID NO: 46 - DNA, 24 bp, synthetic construct
  misc_feature 1..24: note = Synthetic
  source 1..24: mol_type = other DNA
cagccttgaaagtatggcttgggc

SEQ ID NO: 47 - DNA, 18 bp, synthetic construct
  misc_feature 1..18: note = Synthetic
  source 1..18: mol_type = other DNA
gcactcgccaaccggaag

SEQ ID NO: 48 - DNA, 23 bp, synthetic construct
  misc_feature 1..23: note = Synthetic
  source 1..23: mol_type = other DNA
gaccagctcacccttacttatgg

SEQ ID NO: 49 - DNA, 23 bp, synthetic construct
  misc_feature 1..23: note = Synthetic
  source 1..23: mol_type = other DNA
actgaatgccaagggtgcgttga

SEQ ID NO: 50 - DNA, 23 bp, synthetic construct
  misc_feature 1..23: note = Synthetic
  source 1..23: mol_type = other DNA
tcttggaaatccgctgaagagtt

SEQ ID NO: 51 - protein, 31 aa, Mus musculus
MSPWLKWHGPAMARLWGLCLLVLGFWRASLA

SEQ ID NO: 52 - protein, 398 aa, Mus musculus
CPTSCKCSSARIWCTEPSPGIVAFPRLEPNSVDPENITEILIANQKRLEIINEDDVEAYVGLRNLTIVDSGLKFVAYKAFLKNSNLRHINFTRNKLTSLSRRHFRHLDLSDLILTGNPFTCSCDIMWLKTLQETKSSPDTQDLYCLNESSKNMPLANLQIPNCGLPSARLAAPNLTVEEGKSVTLSCSVGGDPLPTLYWDVGNLVSKHMNETSHTQGSLRITNISSDDSGKQISCVAENLVGEDQDSVNLTVHFAPTITFLESPTSDHHWCIPFTVRGNPKPALQWFYNGAILNESKYICTKIHVTNHTEYHGCLQLDNPTHMNNGDYTLMAKNEYGKDERQISAHFMGRPGVDYETNPNYPEVLYEDWTTPTDIGDTTNKSNEIPSTDVADQSNREH

SEQ ID NO: 53 - protein, 24 aa, Mus musculus
LSVYAVVVIASVVGFCLLVMLLLL

SEQ ID NO: 54 - protein, 368 aa, Mus musculus
KLARHSKFGMKGPASVISNDDDSASPLHHISNGSNTPSSSEGGPDAVIIGMTKIPVIENPQYFGITNSQLKPDTFVQHIKRHNIVLKRELGEGAFGKVFLAECYNLCPEQDKILVAVKTLKDASDNARKDFHREAELLTNLQHEHIVKFYGVCVEGDPLIMVFEYMKHGDLNKFLRAHGPDAVLMAEGNPPTELTQSQMLHIAQQIAAGMVYLASQHFVHRDLATRNCLVGENLLVKIGDFGMSRDVYSTDYYRVGGHTMLPIRWMPPESIMYRKFTTESDVWSLGVVLWEIFTYGKQPWYQLSNNEVIECITQGRVLQRPRTCPQEVYELMLGCWQREPHTRKNIKSIHTLLQNLAKASPVYLDILG

SEQ ID NO: 55 - protein, 31 aa, Rattus norvegicus
MSPWPRWHGPAMARLWGLCLLVLGFWRASLA

SEQ ID NO: 56 - protein, 398 aa, Rattus norvegicus
CPMSCKCSTTRIWCTEPSPGIVAFPRLEPNSIDPENITEILIANQKRLEIINEDDVEAYVGLKNLTIVDSGLKFVAYKAFLKNGNLRHINFTRNKLTSLSRRHFRHLDLSDLILTGNPFTCSCDIMWLKTLQETKSSPDTQDLYCLNESSKNTPLANLQIPNCGLPSARLAAPNLTVEEGKSVTISCSVGGDPLPTLYWDVGNLVSKHMNETSHTQGSLRITNISSDDSGKQISCVAENLVGEDQDSVNLTVHFAPTITFLESPTSDHHWCIPFTVRGNPKPALQWFYNGAILNESKYICTKIHVTNHTEYHGCLQLDNPTHMNNGDYTLMAKNEYGKDERQISAHFMGRPGVDYETNPNYPEVLYEDWTTPTDIGDTTNKSNEIPSTDVADQTNREH

SEQ ID NO: 57 - protein, 24 aa, Rattus norvegicus
LSVYAVVVIASVVGFCLLVMLLLL

SEQ ID NO: 58 - protein, 368 aa, Rattus norvegicus
KLARHSKFGMKGPASVISNDDDSASPLHHISNGSNTPSSSEGGPDAVIIGMTKIPVIENPQYFGITNSQLKPDTFVQHIKRHNIVLKRELGEGAFGKVFLAECYNLCPEQDKILVAVKTLKDASDNARKDFHREAELLTNLQHEHIVKFYGVCVEGDPLIMVFEYMKHGDLNKFLRAHGPDAVLMAEGNPPTELTQSQMLHIAQQIAAGMVYLASQHFVHRDLATRNCLVGENLLVKIGDFGMSRDVYSTDYYRVGGHTMLPIRWMPPESIMYRKFTTESDVWSLGVVLWEIFTYGKQPWYQLSNNEVIECITQGRVLQRPRTCPQEVYELMLGCWQREPHTRKNIKNIHTLLQNLAKASPVYLDILG

SEQ ID NO: 59 - protein, 31 aa, Homo sapiens
MSSWIRWHGPAMARLWGFCWLVVGFWRAAFA

SEQ ID NO: 60 - protein, 399 aa, Homo sapiens
CPTSCKCSASRIWCSDPSPGIVAFPRLEPNSVDPENITEIFIANQKRLEIINEDDVEAYVGLRNLTIVDSGLKFVAHKAFLKNSNLQHINFTRNKLTSLSRKHFRHLDLSELILVGNPFTCSCDIMWIKTLQEAKSSPDTQDLYCLNESSKNIPLANLQIPNCGLPSANLAAPNLTVEEGKSITLSCSVAGDPVPNMYWDVGNLVSKHMNETSHTQGSLRITNISSDDSGKQISCVAENLVGEDQDSVNLTVHFAPTITFLESPTSDHHWCIPFTVKGNPKPALQWFYNGAILNESKYICTKIHVTNHTEYHGCLQLDNPTHMNNGDYTLIAKNEYGKDEKQISAHFMGWPGIDDGANPNYPDVIYEDYGTAANDIGDTTNRSNEIPSTDVTDKTGREH

SEQ ID NO: 61 - protein, 24 aa, Homo sapiens
LSVYAVVVIASVVGFCLLVMLFLL

SEQ ID NO: 62 - protein, 384 aa, Homo sapiens
KLARHSKFGMKDFSWFGFGKVKSRQGVGPASVISNDDDSASPLHHISNGSNTPSSSEGGPDAVIIGMTKIPVIENPQYFGITNSQLKPDTFVQHIKRHNIVLKRELGEGAFGKVFLAECYNLCPEQDKILVAVKTLKDASDNARKDFHREAELLTNLQHEHIVKFYGVCVEGDPLIMVFEYMKHGDLNKFLRAHGPDAVLMAEGNPPTELTQSQMLHIAQQIAAGMVYLASQHFVHRDLATRNCLVGENLLVKIGDFGMSRDVYSTDYYRVGGHTMLPIRWMPPESIMYRKFTTESDVWSLGVVLWEIFTYGKQPWYQLSNNEVIECITQGRVLQRPRTCPQEVYELMLGCWQREPHMRKNIKGIHTLLQNLAKASPVYLDILG

SEQ ID NO: 63 - DNA, 93 bp, Mus musculus
  source 1..93: mol_type = other DNA
atgtcgccctggctgaagtggcatggacccgccatggcgcggctctggggcttatgcctgctggtcttgggcttctggagggcctctctcgcc

SEQ ID NO: 64 - DNA, 1194 bp, Mus musculus
  source 1..1194: mol_type = other DNA
tgcccgacgtcctgcaaatgcagttccgctaggatttggtgtactgagccttctccaggcatcgtggcattcccgaggttggaacctaacagcgttgacccggagaacatcacggaaattctcattgcaaaccagaaaaggctagaaatcatcaatgaagatgacgttgaagcttacgtggggctgagaaaccttacaattgtggattccggcttaaagtttgtggcttacaaagcgtttctgaaaaacagcaacctgcggcacataaatttcacacgaaacaagctgacgagtttgtccaggagacatttccgccaccttgacttgtctgacctgatcctgacgggtaatccgttcacgtgctcctgcgacatcatgtggctcaagactctccaggagactaaatccagccccgacactcaggatttgtactgcctcaatgagagcagcaagaacatgcccctggcgaacctgcagatacccaattgtggtctgccatctgcacgtctggctgctcctaacctcaccgtggaggaaggaaagtctgtgaccctttcctgcagtgtggggggtgacccactccccaccttgtactgggacgttgggaatttggtttccaagcacatgaatgaaacaagccacacacagggctccttaaggataacgaacatttcatctgatgacagtggaaagcaaatctcttgtgtggcagaaaaccttgtaggagaagatcaagattctgtgaacctcactgtgcattttgcgccaactatcacgtttctcgagtctccaacctcagatcaccactggtgcattccattcactgtgagaggcaaccccaagcctgcgcttcagtggttctacaatggggccatactgaatgagtccaagtacatctgtactaagatccacgtcaccaatcacacggagtaccatggctgcctccagctggataaccccactcatatgaataacggagactacaccctgatggccaagaacgagtatgggaaggatgagagacagatctccgctcacttcatgggccggcctggagtcgactacgagacaaacccaaattaccctgaagtcctctatgaagactggaccacgccaactgacattggggatactacgaacaaaagtaatgaaatcccctccacggatgttgctgaccaaagcaatcgggagcat

SEQ ID NO: 65 - DNA, 72 bp, Mus musculus
  source 1..72: mol_type = other DNA
ctctcggtctatgccgtggtggtgattgcatctgtggtgggattctgcctgctggtgatgttgctcctgctc

SEQ ID NO: 66 - DNA, 1104 bp, Mus musculus
  source 1..1104: mol_type = other DNA
aagttggcgagacattccaagtttggcatgaaaggcccagcttcggtcatcagcaacgacgatgactctgccagccccctccaccacatctccaatgggagtaacactccatcttcttcggagggcggtcccgacgctgtcattattggaatgaccaagattcctgttattgaaaacccccagtactttggcatcaccaacagtcagctcaagccagacacatttgttcagcatatcaagagacacaacatcgttctgaagagggaacttggggaaggagccttcgggaaagttttccttgccgagtgctacaacctctgcccagagcaggataagatcctggtggctgtgaagacgctgaaggacgccagcgacaatgcacgcaaggactttcatcgggaagctgagctgctgaccaacctccagcacgagcacattgtcaagttctacggtgtctgtgtggagggcgacccactcatcatggtctttgagtacatgaagcacggggacctcaacaagttccttagggcacacgggcccgacgcagtgctgatggcagagggtaacccgcccacagagctgacgcagtcgcagatgctgcacatcgctcagcaaatcgcagcaggtatggtctacctggcgtcccaacactttgtgcaccgtgacctggccacccggaactgcctggtgggagagaacctgctggtgaaaattggggactttgggatgtcccgagatgtgtacagcaccgactactatcgggtcggtggccacacaatgttgcccatccgatggatgcctccagagagcatcatgtacaggaaattcaccaccgagagcgacgtctggagcctgggcgttgtgttgtgggagatcttcacctacggcaagcagccctggtatcagctatcgaacaatgaggtgatagagtgcatcacccagggaagagtccttcagcggcctcgaacgtgtccccaggaggtgtatgagctcatgcttggatgctggcagcgggaaccacacacccggaagaacatcaagagcatccacaccctccttcagaacttggccaaggcatctcccgtctacctggatatcctaggc

SEQ ID NO: 67 - DNA, 93 bp, Rattus norvegicus
  source 1..93: mol_type = other DNA
atgtcgccctggccgaggtggcatggacccgccatggcgcggctctggggcttatgcttgctggtcttgggcttctggagggcttctcttgcc

SEQ ID NO: 68 - DNA, 1194 bp, Rattus norvegicus
  source 1..1194: mol_type = other DNA
tgccccatgtcctgcaaatgcagcaccactaggatttggtgtaccgagccttctcctggcatcgtggcatttccgaggttggaacctaacagcattgacccagagaacatcaccgaaattctcattgcaaaccagaaaaggttagaaatcatcaatgaagatgatgtcgaagcttacgtggggctgaaaaaccttacaattgtggattccggcttaaagtttgtggcttacaaggcgtttctgaagaacggcaacctgcggcacatcaatttcactcgaaacaagctgacgagtttgtccaggagacatttccgccaccttgacttgtctgacctgatcctgacgggtaatccgttcacgtgttcctgtgacatcatgtggctcaagactctccaggagacgaaatccagccccgacactcaggatttgtattgcctcaatgagagcagcaagaatacccctctggcgaacctgcagattcccaattgtggtctgccgtctgcacgtctggccgctcctaacctcacggtggaggaagggaagtctgtgaccatttcctgcagcgtcgggggtgacccgctccccaccttgtactgggacgttgggaatttggtttccaaacacatgaatgaaacaagccacacacagggctccttaaggataacaaacatttcatcggatgacagtgggaaacaaatctcttgtgtggcagaaaacctcgttggagaagatcaagactctgtgaacctcactgtgcattttgcaccaaccatcacatttctcgaatctccaacctcagaccaccactggtgcatcccattcactgtgagaggcaaccccaagccagcacttcagtggttctacaacggagccatactgaatgaatccaagtacatctgtaccaaaatacacgtcaccaatcacacggagtaccacggctgcctccagctggataaccccactcatatgaataatggagactacaccctaatggccaagaatgaatatgggaaggacgagagacagatttctgctcacttcatgggccggcctggagttgactatgagacaaacccaaattaccctgaagtcctctatgaagactggaccacgccaactgacatcggggatactacaaacaaaagtaatgagatcccctccacggatgttgctgaccaaaccaatcgggagcat

SEQ ID NO: 69 - DNA, 72 bp, Rattus norvegicus
  source 1..72: mol_type = other DNA
ctctcggtctatgccgtggtggtgattgcctctgtggtaggattctgcctgctggtgatgctgcttctgctc

SEQ ID NO: 70 - DNA, 1104 bp, Rattus norvegicus
  source 1..1104: mol_type = other DNA
aagttggcgagacattccaagtttggcatgaaaggcccagcttccgtcatcagcaacgacgatgactctgccagccctctccaccacatctccaacgggagcaacactccgtcttcttcggagggcgggcccgatgctgtcatcattgggatgaccaagatccctgtcattgaaaacccccagtacttcggtatcaccaacagccagctcaagccggacacatttgttcagcacatcaagagacacaacatcgttctgaagagggagcttggagaaggagcctttgggaaagttttcctagcggagtgctataacctctgccccgagcaggataagatcctggtggccgtgaagacgctgaaggacgccagcgacaatgctcgcaaggactttcatcgcgaagccgagctgctgaccaacctccagcacgagcacattgtcaagttctacggtgtctgtgtggagggcgacccactcatcatggtctttgagtacatgaagcacggggacctcaacaagttccttagggcacacgggccagatgcagtgctgatggcagagggtaacccgcccaccgagctgacgcagtcgcagatgctgcacatcgctcagcaaatcgcagcaggcatggtctacctggcatcccaacacttcgtgcaccgagacctggccacccggaactgcttggtaggagagaacctgctggtgaaaattggggacttcgggatgtcccgggatgtatacagcaccgactactaccgggttggtggccacacaatgttgcccatccgatggatgcctccagagagcatcatgtacaggaaattcaccaccgagagtgacgtctggagcctgggagttgtgttgtgggagatcttcacctacggcaagcagccctggtatcagctatcaaacaacgaggtgatagaatgcatcacccagggcagagtccttcagcggcctcgcacgtgtccccaggaggtgtacgagctgatgctgggatgctggcagcgggaaccacacacaaggaagaacatcaagaacatccacacactccttcagaacttggcgaaggcgtcgcccgtctacctggacatcctaggc

SEQ ID NO: 71 - DNA, 93 bp, Homo sapiens
  source 1..93: mol_type = other DNA
atgtcgtcctggataaggtggcatggacccgccatggcgcggctctggggcttctgctggctggttgtgggcttctggagggccgctttcgcc

SEQ ID NO: 72 - DNA, 1197 bp, Homo sapiens
  source 1..1197: mol_type = other DNA
tgtcccacgtcctgcaaatgcagtgcctctcggatctggtgcagcgacccttctcctggcatcgtggcatttccgagattggagcctaacagtgtagatcctgagaacatcaccgaaattttcatcgcaaaccagaaaaggttagaaatcatcaacgaagatgatgttgaagcttatgtgggactgagaaatctgacaattgtggattctggattaaaatttgtggctcataaagcatttctgaaaaacagcaacctgcagcacatcaattttacccgaaacaaactgacgagtttgtctaggaaacatttccgtcaccttgacttgtctgaactgatcctggtgggcaatccatttacatgctcctgtgacattatgtggatcaagactctccaagaggctaaatccagtccagacactcaggatttgtactgcctgaatgaaagcagcaagaatattcccctggcaaacctgcagatacccaattgtggtttgccatctgcaaatctggccgcacctaacctcactgtggaggaaggaaagtctatcacattatcctgtagtgtggcaggtgatccggttcctaatatgtattgggatgttggtaacctggtttccaaacatatgaatgaaacaagccacacacagggctccttaaggataactaacatttcatccgatgacagtgggaagcagatctcttgtgtggcggaaaatcttgtaggagaagatcaagattctgtcaacctcactgtgcattttgcaccaactatcacatttctcgaatctccaacctcagaccaccactggtgcattccattcactgtgaaaggcaaccccaaaccagcgcttcagtggttctataacggggcaatattgaatgagtccaaatacatctgtactaaaatacatgttaccaatcacacggagtaccacggctgcctccagctggataatcccactcacatgaacaatggggactacactctaatagccaagaatgagtatgggaaggatgagaaacagatttctgctcacttcatgggctggcctggaattgacgatggtgcaaacccaaattatcctgatgtaatttatgaagattatggaactgcagcgaatgacatcggggacaccacgaacagaagtaatgaaatcccttccacagacgtcactgataaaaccggtcgggaacat

SEQ ID NO: 73 - DNA, 72 bp, Homo sapiens
  source 1..72: mol_type = other DNA
ctctcggtctatgctgtggtggtgattgcgtctgtggtgggattttgccttttggtaatgctgtttctgctt

SEQ ID NO: 74 - DNA, 1152 bp, Homo sapiens
  source 1..1152: mol_type = other DNA
aagttggcaagacactccaagtttggcatgaaagatttctcatggtttggatttgggaaagtaaaatcaagacaaggtgttggcccagcctccgttatcagcaatgatgatgactctgccagcccactccatcacatctccaatgggagtaacactccatcttcttcggaaggtggcccagatgctgtcattattggaatgaccaagatccctgtcattgaaaatccccagtactttggcatcaccaacagtcagctcaagccagacacatttgttcagcacatcaagcgacataacattgttctgaaaagggagctaggcgaaggagcctttggaaaagtgttcctagctgaatgctataacctctgtcctgagcaggacaagatcttggtggcagtgaagaccctgaaggatgccagtgacaatgcacgcaaggacttccaccgtgaggccgagctcctgaccaacctccagcatgagcacatcgtcaagttctatggcgtctgcgtggagggcgaccccctcatcatggtctttgagtacatgaagcatggggacctcaacaagttcctcagggcacacggccctgatgccgtgctgatggctgagggcaacccgcccacggaactgacgcagtcgcagatgctgcatatagcccagcagatcgccgcgggcatggtctacctggcgtcccagcacttcgtgcaccgcgatttggccaccaggaactgcctggtcggggagaacttgctggtgaaaatcggggactttgggatgtcccgggacgtgtacagcactgactactacagggtcggtggccacacaatgctgcccattcgctggatgcctccagagagcatcatgtacaggaaattcacgacggaaagcgacgtctggagcctgggggtcgtgttgtgggagattttcacctatggcaaacagccctggtaccagctgtcaaacaatgaggtgatagagtgtatcactcagggccgagtcctgcagcgaccccgcacgtgcccccaggaggtgtatgagctgatgctggggtgctggcagcgagagccccacatgaggaagaacatcaagggcatccataccctccttcagaacttggccaaggcatctccggtctacctggacattctaggc

SEQ ID NO: 75 - protein, 822 aa, Homo sapiens
  REGION 1..31: note = MISC_FEATURE - Signal Peptide
  REGION 32..430: note = MISC_FEATURE - Extracellular Domain
  REGION 431..454: note = MISC_FEATURE - Transmembrane Domain
  REGION 455..822: note = MISC_FEATURE - Cytoplasmic Domain
MSSWIRWHGPAMARLWGFCWLVVGFWRAAFACPTSCKCSASRIWCSDPSPGIVAFPRLEPNSVDPENITEIFIANQKRLEIINEDDVEAYVGLRNLTIVDSGLKFVAHKAFLKNSNLQHINFTRNKLTSLSRKHFRHLDLSELILVGNPFTCSCDIMWIKTLQEAKSSPDTQDLYCLNESSKNIPLANLQIPNCGLPSANLAAPNLTVEEGKSITLSCSVAGDPVPNMYWDVGNLVSKHMNETSHTQGSLRITNISSDDSGKQISCVAENLVGEDQDSVNLTVHFAPTITFLESPTSDHHWCIPFTVKGNPKPALQWFYNGAILNESKYICTKIHVTNHTEYHGCLQLDNPTHMNNGDYTLIAKNEYGKDEKQISAHFMGWPGIDDGANPNYPDVIYEDYGTAANDIGDTTNRSNEIPSTDVTDKTGREHLSVYAVVVIASVVGFCLLVMLFLLKLARHSKFGMKGPASVISNDDDSASPLHHISNGSNTPSSSEGGPDAVIIGMTKIPVIENPQYFGITNSQLKPDTFVQHIKRHNIVLKRELGEGAFGKVFLAECYNLCPEQDKILVAVKTLKDASDNARKDFHREAELLTNLQHEHIVKFYGVCVEGDPLIMVFEYMKHGDLNKFLRAHGPDAVLMAEGNPPTELTQSQMLHIAQQIAAGMVYLASQHFVHRDLATRNCLVGENLLVKIGDFGMSRDVYSTDYYRVGGHTMLPIRWMPPESIMYRKFTTESDVWSLGVVLWEIFTYGKQPWYQLSNNEVIECITQGRVLQRPRTCPQEVYELMLGCWQREPHMRKNIKGIHTLLQNLAKASPVYLDILG

SEQ ID NO: 76 - DNA, 8498 bp, Homo sapiens
  source 1..8498: mol_type = other DNA
cctcgaggtgcataccggacccccattcgcatctaacaaggaatctgcgccccagagagtcccgggagcgccgccggtcggtgcccggcgcgccgggccatgcagcgacggccgccgcggagctccgagcagcggtagcgcccccctgtaaagcggttcgctatgccggggccactgtgaaccctgccgcctgccggaacactcttcgctccggaccagctcagcctctgataagctggactcggcacgcccgcaacaagcaccgaggagttaagagagccgcaagcgcagggaaggcctccccgcacgggtgggggaaagcggccggtgcagcgcggggacaggcactcgggctggcactggctgctagggatgtcgtcctggataaggtggcatggacccgccatggcgcggctctggggcttctgctggctggttgtgggcttctggagggccgctttcgcctgtcccacgtcctgcaaatgcagtgcctctcggatctggtgcagcgacccttctcctggcatcgtggcatttccgagattggagcctaacagtgtagatcctgagaacatcaccgaaattttcatcgcaaaccagaaaaggttagaaatcatcaacgaagatgatgttgaagcttatgtgggactgagaaatctgacaattgtggattctggattaaaatttgtggctcataaagcatttctgaaaaacagcaacctgcagcacatcaattttacccgaaacaaactgacgagtttgtctaggaaacatttccgtcaccttgacttgtctgaactgatcctggtgggcaatccatttacatgctcctgtgacattatgtggatcaagactctccaagaggctaaatccagtccagacactcaggatttgtactgcctgaatgaaagcagcaagaatattcccctggcaaacctgcagatacccaattgtggtttgccatctgcaaatctggccgcacctaacctcactgtggaggaaggaaagtctatcacattatcctgtagtgtggcaggtgatccggttcctaatatgtattgggatgttggtaacctggtttccaaacatatgaatgaaacaagccacacacagggctccttaaggataactaacatttcatccgatgacagtgggaagcagatctcttgtgtggcggaaaatcttgtaggagaagatcaagattctgtcaacctcactgtgcattttgcaccaactatcacatttctcgaatctccaacctcagaccaccactggtgcattccattcactgtgaaaggcaaccccaaaccagcgcttcagtggttctataacggggcaatattgaatgagtccaaatacatctgtactaaaatacatgttaccaatcacacggagtaccacggctgcctccagctggataatcccactcacatgaacaatggggactacactctaatagccaagaatgagtatgggaaggatgagaaacagatttctgctcacttcatgggctggcctggaattgacgatggtgcaaacccaaattatcctgatgtaatttatgaagattatggaactgcagcgaatgacatcggggacaccacgaacagaagtaatgaaatcccttccacagacgtcactgataaaaccggtcgggaacatctctcggtctatgctgtggtggtgattgcgtctgtggtgggattttgccttttggtaatgctgtttctgcttaagttggcaagacactccaagtttggcatgaaaggcccagcctccgttatcagcaatgatgatgactctgccagcccactccatcacatctccaatgggagtaacactccatcttcttcggaaggtggcccagatgctgtcattattggaatgaccaagatccctgtcattgaaaatccccagtactttggcatcaccaacagtcagctcaagccagacacatttgttcagcacatcaagcgacataacattgttctgaaaagggagctaggcgaaggagcctttggaaaagtgttcctagctgaatgctataacctctgtcctgagcaggacaagatcttggtggcagtgaagaccctgaaggatgccagtgacaatgcacgcaaggacttccaccgtgaggccgagctcctgaccaacctccagcatgagcacatcgtcaagttctatggcgtctgcgtggagggcgaccccctcatcatggtctttgagtacatgaagcatggggacctcaacaagttcctcagggcacacggccctgatgccgtgctgatggctgagggcaacccgcccacggaactgacgcagtcgcagatgctgcatatagcccagcagatcgccgcgggcatggtctacctggcgtcccagcacttcgtgcaccgcgatttggccaccaggaactgcctggtcggggagaacttgctggtgaaaatcggggactttgggatgtcccgggacgtgtacagcactgactactacagggtcggtggccacacaatgctgcccattcgctggatgcctccagagagcatcatgtacaggaaattcacgacggaaagcgacgtctggagcctgggggtcgtgttgtgggagattttcacctatggcaaacagccctggtaccagctgtcaaacaatgaggtgatagagtgtatcactcagggccgagtcctgcagcgaccccgcacgtgcccccaggaggtgtatgagctgatgctggggtgctggcagcgagagccccacatgaggaagaacatcaagggcatccataccctccttcagaacttggccaaggcatctccggtctacctggacattctaggctagggcccttttccccagaccgatccttcccaacgtactcctcagacgggctgagaggatgaacatcttttaactgccgctggaggccaccaagctgctctccttcactctgacagtattaacatcaaagactccgagaagctctcgagggaagcagtgtgtacttcttcatccatagacacagtattgacttctttttggcattatctctttctctctttccatctcccttggttgttcctttttctttttttaaattttctttttcttttttttttcgtcttccctgcttcacgattcttaccctttcttttgaatcaatctggcttctgcattactattaactctgcatagacaaaggccttaacaaacgtaatttgttatatcagcagacactccagtttgcccaccacaactaacaatgccttgttgtattcctgcctttgatgtggatgaaaaaaagggaaaacaaatatttcacttaaactttgtcacttctgctgtacagatatcgagagtttctatggattcacttctatttatttattattattactgttcttattgtttttggatggcttaagcctgtgtataaaaaagaaaacttgtgttcaatctgtgaagcctttatctatgggagattaaaaccagagagaaagaagatttattatgaaccgcaatatgggaggaacaaagacaaccactgggatcagctggtgtcagtccctacttaggaaatactcagcaactgttagctgggaagaatgtattcggcaccttcccctgaggacctttctgaggagtaaaaagactactggcctctgtgccatggatgattcttttcccatcaccagaaatgatagcgtgcagtagagagcaaagatggcttccgtgagacacaagatggcgcatagtgtgctcggacacagttttgtcttcgtaggttgtgatgatagcactggtttgtttctcaagcgctatccacagaacctttgtcaacttcagttgaaaagaggtggattcatgtccagagctcatttcggggtcaggtgggaaagccaagaacttggaaaagataagacaagctataaattcggaggcaagtttcttttacaatgaacttttcagatctcacttccctccgacccctaacttccatgcccacccgtccttttaactgtgcaagcaaaattgtgcatggtcttcgtcgattaataccttgtgtgcagacactactgctccagacgtcgtttccctgataggtagagcagatccataaaaaggtatgacttatacaattaggggaagctaatggagtttattagctgagtatcaatgtctctgcgttgtacggtggtgatgggttttaatgaatatggaccctgaagcctggaaatcctcatccacgtcgaacccacaggactgtgggaagggcagaatcaatccctaagggaaaggaaacctcaccctgagggcatcacatgcactcatgttcagtgtacacaggtcaagtcccttgctctgggctctagttgggagagtggtttcattccaagtgtactccattgtcagtatgctgtttttgtttccttcactccattcaaaaagtcaaaatacaaaatttggcacagcatgccaacgggaggctgtgcccagaccaagcactggaagtgtgcttctaggcatagtcattggttttgcaaaaagagggctcaaatttaaatagaaatttacagctatttgaatggtcagatataccaagaaagaaaaatatttctgttcctcaagaaaacttgctaccctctgtgaggggaattttgctaaacttgacatctttataacatgagccagattgaaagggagtgattttcattcatcttaggtcatgttatttcatatttgtttctgaaggtgcgatagctctgttttaggttttgcttgcgcctgttaattactggaacaccttatttttcattaaaggctttgaaagccaattctcaaaaattcaaaagtgcaaattaacagaacaaaaggaaatccagtagcaactgcagtcaagcgagggagttgacaagataaaccttacgtccattcaagttatatgctggcctatgagagatgagagttgggtcgtttgttctctttgttgatgattttaaaaaaaccctctagaatacacataataacataatgaaagccatatctccatgatatatatgtgcacatatatatacatacatgtgcatgtatgtatcatattaaggacccatggtactcttaaaacactgtagaactctgtgacgcagtaaggaaggggcagatttgtacaaaaacttttctagattccatcagcaaaaaccaacacaggtttgtcacgctgcatgtctggccagctaatctcgggggaaaagctacaagttatttattttattttaagagaataaagtaggtaataatttaagggatcaaattcaaggaggaatgtgcaattttagagcaaagatttgtttaaggcaaatgagactttgggagcatcccattccagttttgtcttttttttctctgaaagaaaaaagcaaaaaataaaataaaattccacttataccttctgacaagtccctaaaggtcttgaaataaaaggttctatgcaagtgcaaagttttatagttatttttattgctgattattactattactatctctgttgtcttaagagtatgtgctgatttcagagacatctcaaattgaaagaatatcagattgcttttaaagtagctgaacgagccacagaatatctgaaattattcattgttgttcctccaccaccccctttctcatggtctgatttttagaagagtggcatcctcgttctaaaatgtaatgatcaccaaatacggccttccatcaaatttgtgaaaactacaacagtataacagtgacaaacctaattctctagcccaaacctggtctgacaatcatttccatttagaagtcattgaatagttttccaaacactttccatgtgtgttagcaaattattcctattttgtgtagatgaggacgttgagactcagagacattcagaggcacgctagaggtctccagcctagcttccagcaccattgggactgaatccaagtactctcactctgaacttcgtggttctgtccactagagactctaatatgcaaacaagcagttcaggaaagaaagcatgctaacacattcatgaagcagtatatgaagttagaagaacaaaaggaaatacaggagatgacaagcaactgagatattgtgatatataatcatgctcttagcttcagctaaattcagctaaattcttgtacactgaaccaatgtcataatcaggcttatttagaaaacactttgaactatgctataaaagattatatcagaattcatattatacatgtgttcacatcagcgctacctgtgatgttttcatgtatttatgtatgtgttataaatacttgatttatacatatacaaatgcacatacgtagtgtgtttgtgtgtttatgtataaatttataggcacacaataatagaggtaattataagtaggatgcggtatgaataatttgcttaaaatatgctaaataaccaaaactgtttaacgtcatgttgctgttagtgcttccatactccacgtgggtaggactacatcacacttttcaactctgtgcagtactgcatgggtggaagacatatttaagataatgtgcttcccaaaacaactgaataaaagccatcccactacattgagtgctttctctggctccttgcaaagaaagatactttttgtaatggtccaggaaaggaacattgctttctttttgtctttcagcacatttgtattatgctcaccttgtctctgtctcactgtgacccctttacacttgagttcagagttcaagcattccaaatataaattggaatgttggcagcccagtggcttgaaggccaatgatgagcagtccaagaccccacagcgagatgagcaactcttaggaattcccacatcctagagtgaatgcaccaactaacagtatagaatgctgtccttttcaaagcgtcctaacagcaggattacctggtcaagtatggactttctttgaatctttcttttcacaaattggactgcctgtaataccaataacattgttgtatctaactaaataaatgactgcatatacacacataccctcaattctcttgcttccccattttctttttcatcccctgtctcaggacttttattttcaatgttgacctttggtttggccatatatcactgttataggaaatctcatgagaggaatggctagtgacccaactctccaaatgtctaagttagtagttacagctgattttttatgatgcataattggaatgtggagcctctgaggttgtgatagcttgtacatgaatttcaaatgtcattctaaagaatgaggggtgggagggatttatagttagaaacgacagtgcaggaaggggtattttcttgttgtcagggctggaatgaatcactgctgctcaagtcaaaggttcttgaatatccttagtttttgcatttcccctccttttcctttgacctttatttatttaattatgtatttatttatttatttatatacttttgctccattcagcacaaacacaaagcaaagcaaaaaaaaaaatatatatatatatatctgtatatgtgttgtaggcaaaacactgtgaatttcacaacaaccaccaccaagcaactattttgccatcttaacatacatctcaggagacgaaatgagaaaagatggggatgtcattttttagtctatgcgtttgaggccaggtccatgtttatttatttctttagtctatgcattaatgaaaatgatcctgagtggaggttagctgaacgttcaatgtactggagcaagcatcataaaagctgctagtagccatgtgtttgaacaggaaaaatattacagaaaatgaaatgtaaaggcctatatcttgcagcttgtatatcttactattgcttaaaaaatgtataaagcagctggaaatgttttaaatacaaggtctttgaattaaatgtggattttaaatatgtaatcccttgacaaatgaccaaattatggtgaactattgctccctgcgttctttgatcattacctatgacttacaaatctgcctggagatgtggacattctgcatttgcttctgtatctggagagatgtttgtatatatccaggccgtatacacacacatttccatatctctctacagatatatttccccttcaatcgtgacctggtatttggaactctccttttcatttggcttatcttccttttaatgtgatgtctctgtgctaatacttaccagttcttgttttgcaatctgttttgaggtccattgctttactaagacccactgcatcttggctgatttcaaagtgacacctgaatacagtgtttaaaaaaaaaaaagttttgtttgtaaatcatgtgaccagcttctctcaacctgacatggaaagtctcttgtactacagtgtatttaataaaaatgatgtcttacaataaataacatactccaaaagagagactaaaaatgaaaaaaaaaaaaaaaaaaaaaaaaa

SEQ ID NO: 77 - DNA, 2469 bp, Homo sapiens
  misc_feature 1..93: note = Signal Peptide
  misc_feature 94..1290: note = Extracellular Domain
  misc_feature 1291..1362: note = Transmembrane Domain
  misc_feature 1363..2466: note = Cytoplasmic Domain
  source 1..2469: mol_type = other DNA
atgtcgtcctggataaggtggcatggacccgccatggcgcggctctggggcttctgctggctggttgtgggcttctggagggccgctttcgcctgtcccacgtcctgcaaatgcagtgcctctcggatctggtgcagcgacccttctcctggcatcgtggcatttccgagattggagcctaacagtgtagatcctgagaacatcaccgaaattttcatcgcaaaccagaaaaggttagaaatcatcaacgaagatgatgttgaagcttatgtgggactgagaaatctgacaattgtggattctggattaaaatttgtggctcataaagcatttctgaaaaacagcaacctgcagcacatcaattttacccgaaacaaactgacgagtttgtctaggaaacatttccgtcaccttgacttgtctgaactgatcctggtgggcaatccatttacatgctcctgtgacattatgtggatcaagactctccaagaggctaaatccagtccagacactcaggatttgtactgcctgaatgaaagcagcaagaatattcccctggcaaacctgcagatacccaattgtggtttgccatctgcaaatctggccgcacctaacctcactgtggaggaaggaaagtctatcacattatcctgtagtgtggcaggtgatccggttcctaatatgtattgggatgttggtaacctggtttccaaacatatgaatgaaacaagccacacacagggctccttaaggataactaacatttcatccgatgacagtgggaagcagatctcttgtgtggcggaaaatcttgtaggagaagatcaagattctgtcaacctcactgtgcattttgcaccaactatcacatttctcgaatctccaacctcagaccaccactggtgcattccattcactgtgaaaggcaaccccaaaccagcgcttcagtggttctataacggggcaatattgaatgagtccaaatacatctgtactaaaatacatgttaccaatcacacggagtaccacggctgcctccagctggataatcccactcacatgaacaatggggactacactctaatagccaagaatgagtatgggaaggatgagaaacagatttctgctcacttcatgggctggcctggaattgacgatggtgcaaacccaaattatcctgatgtaatttatgaagattatggaactgcagcgaatgacatcggggacaccacgaacagaagtaatgaaatcccttccacagacgtcactgataaaaccggtcgggaacatctctcggtctatgctgtggtggtgattgcgtctgtggtgggattttgccttttggtaatgctgtttctgcttaagttggcaagacactccaagtttggcatgaaaggcccagcctccgttatcagcaatgatgatgactctgccagcccactccatcacatctccaatgggagtaacactccatcttcttcggaaggtggcccagatgctgtcattattggaatgaccaagatccctgtcattgaaaatccccagtactttggcatcaccaacagtcagctcaagccagacacatttgttcagcacatcaagcgacataacattgttctgaaaagggagctaggcgaaggagcctttggaaaagtgttcctagctgaatgctataacctctgtcctgagcaggacaagatcttggtggcagtgaagaccctgaaggatgccagtgacaatgcacgcaaggacttccaccgtgaggccgagctcctgaccaacctccagcatgagcacatcgtcaagttctatggcgtctgcgtggagggcgaccccctcatcatggtctttgagtacatgaagcatggggacctcaacaagttcctcagggcacacggccctgatgccgtgctgatggctgagggcaacccgcccacggaactgacgcagtcgcagatgctgcatatagcccagcagatcgccgcgggcatggtctacctggcgtcccagcacttcgtgcaccgcgatttggccaccaggaactgcctggtcggggagaacttgctggtgaaaatcggggactttgggatgtcccgggacgtgtacagcactgactactacagggtcggtggccacacaatgctgcccattcgctggatgcctccagagagcatcatgtacaggaaattcacgacggaaagcgacgtctggagcctgggggtcgtgttgtgggagattttcacctatggcaaacagccctggtaccagctgtcaaacaatgaggtgatagagtgtatcactcagggccgagtcctgcagcgaccccgcacgtgcccccaggaggtgtatgagctgatgctggggtgctggcagcgagagccccacatgaggaagaacatcaagggcatccataccctccttcagaacttggccaaggcatctccggtctacctggacattctaggctag

SEQ ID NO: 78 - DNA, 354 bp, synthetic construct
  misc_feature 1..354: note = Synthetic
  source 1..354: mol_type = other DNA
caggtgcagctggtggagtctgggggaggcgtggtccagcctgggaggtccctgagactctcctgtgcagcctctggattcagcttcagtagctttggcatgcactgggtccgccaggctccaggcaagggactggagtgggtgtcagttatatcatatgatggaattaatacatactatacagactccgtgaagggccgattcaccatctccagagacaattccaagaacacgctgtatctgcaaatgaacggcctgagagctgaggacacggctctttattactgtgtgcaagggtcaattggaaccgtttttgaatactggggccagggaaccctggtcaccgtctcctca

SEQ ID NO: 79 - protein, 118 aa, synthetic construct
  REGION 1..118: note = Synthetic
QVQLVESGGGVVQPGRSLRLSCAASGFSFSSFGMHWVRQAPGKGLEWVSVISYDGINTYYTDSVKGRFTISRDNSKNTLYLQMNGLRAEDTALYYCVQGSIGTVFEYWGQGTLVTVSS

SEQ ID NO: 80 - DNA, 24 bp, synthetic construct
  misc_feature 1..24: note = Synthetic
  source 1..24: mol_type = other DNA
ggattcagcttcagtagctttggc

SEQ ID NO: 81 - protein, 8 aa, synthetic construct
  REGION 1..8: note = Synthetic
GFSFSSFG

SEQ ID NO: 82 - DNA, 24 bp, synthetic construct
  misc_feature 1..24: note = Synthetic
  source 1..24: mol_type = other DNA
atatcatatgatggaattaataca

SEQ ID NO: 83 - protein, 8 aa, synthetic construct
  REGION 1..8: note = Synthetic
ISYDGINT

SEQ ID NO: 84 - DNA, 33 bp, synthetic construct
  misc_feature 1..33: note = Synthetic
  source 1..33: mol_type = other DNA
gtgcaagggtcaattggaaccgtttttgaatac

SEQ ID NO: 85 - protein, 11 aa, synthetic construct
  REGION 1..11: note = Synthetic
VQGSIGTVFEY

SEQ ID NO: 86 - DNA, 321 bp, synthetic construct
  misc_feature 1..321: note = Synthetic
  source 1..321: mol_type = other DNA
gacatccagatgacccagtctccatcctccctgtctgcatctgtaggagacagagtcaccatcacttgccgggcgagtcagggcattagcaattatttagcctggtatcagcagaaaccagggaaagttcctaaactcctgatctatgctgcatccactttacaatcaggggtcccatctcggttcggtggcagtggatctgggacagatttcactctcaccatcagcagcctgcagcctgaagatgttgcaacttattactgtcaaaagtataccagtgccccattcactttcggccctgggaccaaagtggatatcaaa

SEQ ID NO: 87 - protein, 107 aa, synthetic construct
  REGION 1..107: note = Synthetic
DIQMTQSPSSLSASVGDRVTITCRASQGISNYLAWYQQKPGKVPKLLIYAASTLQSGVPSRFGGSGSGTDFTLTISSLQPEDVATYYCQKYTSAPFTFGPGTKVDIK

SEQ ID NO: 88 - DNA, 18 bp, synthetic construct
  misc_feature 1..18: note = Synthetic
  source 1..18: mol_type = other DNA
cagggcattagcaattat

SEQ ID NO: 89 - protein, 6 aa, synthetic construct
  REGION 1..6: note = Synthetic
QGISNY

SEQ ID NO: 90-91 - skipped (2 entries)

SEQ ID NO: 92 - DNA, 27 bp, synthetic construct
  misc_feature 1..27: note = Synthetic
  source 1..27: mol_type = other DNA
caaaagtataccagtgccccattcact

SEQ ID NO: 93 - protein, 9 aa, synthetic construct
  REGION 1..9: note = Synthetic
QKYTSAPFT

SEQ ID NO: 94 - DNA, 366 bp, synthetic construct
  misc_feature 1..366: note = Synthetic
  source 1..366: mol_type = other DNA
gaggtgcagctggtggagtctgggggaggcttggtccagcctggggggtccctaaaactctcctgtacagcctctgggttcaccttcagtggctctgttattcactgggtccgccaggcttccgggaaagggctggagtggattggccgtattagaaacaaggctaacagttacgcgacagcatatggtgcgtcggtgacaggcaggttcaccatctccagagatgattcaaagaacacggcgtatctgcaaatgaacagcctgaaaaccgaggacacggccgtttattactgtactttcccgggtgtagtgggacgaggaggttttgactactggggccagggcaccctggtcaccgtctcctca

SEQ ID NO: 95 - protein, 122 aa, synthetic construct
  REGION 1..122: note = Synthetic
EVQLVESGGGLVQPGGSLKLSCTASGFTFSGSVIHWVRQASGKGLEWIGRIRNKANSYATAYGASVTGRFTISRDDSKNTAYLQMNSLKTEDTAVYYCTFPGVVGRGGFDYWGQGTLVTVSS

SEQ ID NO: 96 - DNA, 24 bp, synthetic construct
  misc_feature 1..24: note = Synthetic
  source 1..24: mol_type = other DNA
gggttcaccttcagtggctctgtt

SEQ ID NO: 97 - protein, 8 aa, synthetic construct
  REGION 1..8: note = Synthetic
GFTFSGSV

SEQ ID NO: 98 - DNA, 30 bp, synthetic construct
  misc_feature 1..30: note = Synthetic
  source 1..30: mol_type = other DNA
attagaaacaaggctaacagttacgcgaca

SEQ ID NO: 99 - protein, 10 aa, synthetic construct
  REGION 1..10: note = Synthetic
IRNKANSYAT

SEQ ID NO: 100 - DNA, 39 bp, synthetic construct
  misc_feature 1..39: note = Synthetic
  source 1..39: mol_type = other DNA
actttcccgggtgtagtgggacgaggaggttttgactac

SEQ ID NO: 101 - protein, 13 aa, synthetic construct
  REGION 1..13: note = Synthetic
TFPGVVGRGGFDY

SEQ ID NO: 102 - DNA, 339 bp, synthetic construct
  misc_feature 1..339: note = Synthetic
  source 1..339: mol_type = other DNA
gacatcgtgatgacccagtctccagactccctggctgtgtctctgggcgagggggccaccatcaactgcatgtccagccagagtgttttattcagctccaacaataagaactacttagcttggtaccaacagaaaccaggacagcctcctaagttgctcttttactgggcatctacccgggaatccggggtccctgaccgattcggtggcagcgggtctgggacagatttctctctcaccatcaacagcctgcagactgaagatgtggcagtttattactgtctccaatattatagtattccgtggacgttcggccaagggaccaaggtggaaatcaaa

SEQ ID NO: 103 - protein, 113 aa, synthetic construct
  REGION 1..113: note = Synthetic
DIVMTQSPDSLAVSLGEGATINCMSSQSVLFSSNNKNYLAWYQQKPGQPPKLLFYWASTRESGVPDRFGGSGSGTDFSLTINSLQTEDVAVYYCLQYYSIPWTFGQGTKVEIK

SEQ ID NO: 104 - DNA, 36 bp, synthetic construct
  misc_feature 1..36: note = Synthetic
  source 1..36: mol_type = other DNA
cagagtgttttattcagctccaacaataagaactac

SEQ ID NO: 105 - protein, 12 aa, synthetic construct
  REGION 1..12: note = Synthetic
QSVLFSSNNKNY

SEQ ID NO: 106-107 - skipped (2 entries)

SEQ ID NO: 108 - DNA, 27 bp, synthetic construct
  misc_feature 1..27: note = Synthetic
  source 1..27: mol_type = other DNA
ctccaatattatagtattccgtggacg

SEQ ID NO: 109 - protein, 9 aa, synthetic construct
  REGION 1..9: note = Synthetic
LQYYSIPWT

SEQ ID NO: 110 - DNA, 381 bp, synthetic construct
  misc_feature 1..381: note = Synthetic
  source 1..381: mol_type = other DNA
gaggtgcagctggtggagtctgggggaggcttggtacagcctggagggtccctgacactctcctgtgcagcctctggattcaatttccgtgattatgaaatgatctgggtccgccagactccagggaaggggctggagtggatttcatacattagtaatagtggttataccatatactacgcagactctgtgaagggccgattcaccatctccagagacaacgccaggaactcaatatatctgcaagtgaacagcctgagagccgaggacacggctgtttattactgttcgagacgtactactatgattcggggcattagggcgtactactattacggtctggacgtctggggccaagggaccacggtcaccgtctcctca

SEQ ID NO: 111 - protein, 127 aa, synthetic construct
  REGION 1..127: note = Synthetic
EVQLVESGGGLVQPGGSLTLSCAASGFNFRDYEMIWVRQTPGKGLEWISYISNSGYTIYYADSVKGRFTISRDNARNSIYLQVNSLRAEDTAVYYCSRRTTMIRGIRAYYYYGLDVWGQGTTVTVSS

SEQ ID NO: 112 - DNA, 24 bp, synthetic construct
  misc_feature 1..24: note = Synthetic
  source 1..24: mol_type = other DNA
ggattcaatttccgtgattatgaa

SEQ ID NO: 113 - protein, 8 aa, synthetic construct
  REGION 1..8: note = Synthetic
GFNFRDYE

SEQ ID NO: 114 - DNA, 24 bp, synthetic construct
  misc_feature 1..24: note = Synthetic
  source 1..24: mol_type = other DNA
attagtaatagtggttataccata

SEQ ID NO: 115 - protein, 8 aa, synthetic construct
  REGION 1..8: note = Synthetic
ISNSGYTI

SEQ ID NO: 116 - DNA, 60 bp, synthetic construct
  misc_feature 1..60: note = Synthetic
  source 1..60: mol_type = other DNA
tcgagacgtactactatgattcggggcattagggcgtactactattacggtctggacgtc

SEQ ID NO: 117 - protein, 20 aa, synthetic construct
  REGION 1..20: note = Synthetic
SRRTTMIRGIRAYYYYGLDV

SEQ ID NO: 118 - DNA, 324 bp, synthetic construct
  misc_feature 1..324: note = Synthetic
  source 1..324: mol_type = other DNA
gacatccagatgacccagtctccatcctccctgtctgcatctgtaggagacagagtcaccatcacttgccgggcaagtcagagcattagcagctatttaaattggtatcagcagaaaccagggaaagcccctaagctcctgatctatgctgcatccagtttgcaaagtggggtcccgtcaaggttcagtggcagtggatctgggacagatttcactctcaccatcagcagtctgcaacctgaagattttgcaacttactactgtcaacagagttacagtacccctccgatcaccttcggccaagggacacgactggagattaaa

SEQ ID NO: 119 - protein, 108 aa, synthetic construct
  REGION 1..108: note = Synthetic
DIQMTQSPSSLSASVGDRVTITCRASQSISSYLNWYQQKPGKAPKLLIYAASSLQSGVPSRFSGSGSGTDFTLTISSLQPEDFATYYCQQSYSTPPITFGQGTRLEIK

SEQ ID NO: 120 - DNA, 18 bp, synthetic construct
  misc_feature 1..18: note = Synthetic
  source 1..18: mol_type = other DNA
cagagcattagcagctat

SEQ ID NO: 121 - protein, 6 aa, synthetic construct
  REGION 1..6: note = Synthetic
QSISSY

SEQ ID NO: 122-123 - skipped (2 entries)

SEQ ID NO: 124 - DNA, 30 bp, synthetic construct
  misc_feature 1..30: note = Synthetic
  source 1..30: mol_type = other DNA
caacagagttacagtacccctccgatcacc

SEQ ID NO: 125 - protein, 10 aa, synthetic construct
  REGION 1..10: note = Synthetic
QQSYSTPPIT